European Patent Specification EP 3 674 313 B1, published November 26, 2025. Title: Novel polypeptide and method of producing IMP using the same. Applicant: CJ CheilJedang Corporation. The sequence listing filed with the application follows.

SEQUENCE LISTING (156 sequences)

SEQ ID NO: 1 - protein, 222 aa, Unknown
  ImpE1
LHAVQEVNDNEEDSLPGSDLGLREQKRLATKHRIEDAATRLVDESSFDKVTIEEICEAAGISRRTFFNYFSTKESAVIGASSEPLTEKQRNDFLNADASNLLQLMVEQIKQHLESSHQSQAIHDRRQRIFADPDVAVRAMAFRKERSRETMELIAQRLREHPEEQRAPELDPETEAMLLSGFIREATWMAISRPDRDCALPVGDRIYRAMELVKNYTKGLEW

SEQ ID NO: 2 - protein, 549 aa, Unknown
  ImpE2
MVAKNSTPSTAGHASAHTAEEFPVANAEMATPSAIDPNHGKKTADNVGIIFAALMLTMLMSSLGQMIFGSALPTIVGELGGVDQMSWVISAFMVTMTIAMPLAGQLGDRMGRKWVYISGISIFVIGSTLGGFANGMGMLITGRAIQGFGAGIMMISSQSIVAEVVSARERGKFMGIMGGVFGVSSVLGPVLGGWFTDGPGWRWGLWINIPLGLLAIIVCAFVLKLRVGEQGFKGFDWMGFAAIAITTSTLILLTTWGGSEYEWTSPTILSMAAVVIVGALLTVFIESRASQPLIPVQLFKNRNMVLTTLAGTVLGLAMMGVLGYMPTYLQMVHTLTPTEAGLMMIPMMVGMIGVSTGVGFIIAKTGNYKYYPIAGLAITAFALWWMSQMTVETSLTGIGVRFLVFGVGLGFVMQVLVLIVQNSFPVSQVGTATAANNFFRQIGSALGASIVGSMFIHNMQNEMATRLPDALASLGKEGAAISQQFQGADAANSLTPHAVAELPDVLRDAILNSYNDGLTPVIGMMVPLAIVAMLILFPLRQERLKETIE

SEQ ID NO: 3 - DNA, 669 bp, Unknown
  ImpE1
ttgcatgctgtgcaagaagttaatgacaatgaagaagactccctccctggcagtgacctcgggttaagggagcagaagcgattggcaaccaagcatcgcatcgaagacgccgcgacacggttggttgatgaatcgagctttgacaaagtaacaattgaagaaatttgcgaagccgccgggatttcccgacgcaccttttttaattatttcagcacgaaagaaagcgccgttattggcgcgtcctcggaaccgttgacggaaaagcaacgcaatgacttcttgaatgctgacgccagcaatctcctgcagctgatggttgagcagatcaaacaacacttggagtcttctcaccagagtcaagcgattcacgaccgtcgtcagcgaatctttgcggatccggatgtcgcggtacgtgcaatggcgtttcgcaaggaacgctcacgggaaaccatggagctaatcgctcaacgtcttcgggagcatcctgaagaacaacgcgccccagaattggatccggaaacagaggcgatgctgctgagcggattcattcgcgaagccacctggatggctatctcacgacccgatcgtgattgtgcactgccagtgggtgaccgcatctatcgcgcgatggaattggtaaagaattacacgaaaggactggaatggtag

SEQ ID NO: 4 - DNA, 1650 bp, Unknown
  ImpE2
atggtagctaaaaactccaccccaagcacggccggccacgccagtgctcacactgcggaagaattcccagtggccaatgctgaaatggcaacgccttcagcaatcgacccaaaccacggtaaaaagaccgcggataacgtcggcattatcttcgctgccttgatgctcaccatgctgatgagctctttggggcagatgattttcggttccgctctgccaaccatcgtcggcgagctcggcggcgtggaccagatgagctgggtaatttcagcatttatggtcaccatgaccattgctatgccactagccggtcagctcggtgaccgcatgggccgcaagtgggtctacatctcaggtatctccattttcgttattggctcgacgctcggtggctttgccaatggcatgggcatgctgatcaccggacgtgcaatccagggcttcggtgccggcatcatgatgatttcctcgcagtcgattgtggctgaggttgtctccgcacgtgagcgcggcaagttcatgggtattatgggcggcgtctttggcgtctcctccgtactgggtccagttctcggtggctggttcaccgatggtcccggttggcgttggggcctgtggatcaacattccactgggtctgctggcaattattgtctgcgctttcgtactgaagctgcgcgtgggcgagcaaggctttaagggctttgactggatgggttttgcggccatcgcaatcacgaccagcaccctgattctgctcaccacttggggcggaagcgaatacgagtggacttccccaactattttgtccatggctgccgtagtcatcgtcggcgcgctgctcaccgtgttcattgagtcgcgtgcatcccagccgctgatcccggttcagctatttaagaaccgcaacatggttttgaccaccctcgccggtactgttttgggtctggccatgatgggcgtgctcggctacatgccaacctacctgcagatggtgcacaccctgacgccaactgaagcaggcttgatgatgatcccgatgatggtcggcatgatcggtgtctccactggtgttggcttcatcatcgctaagaccggcaactacaagtactaccccatcgcgggcctggccatcacggcgtttgctttgtggtggatgtcccagatgaccgttgagacttcattgaccggtatcggagttcgcttccttgtattcggtgtcggcttgggctttgtcatgcaggtactggtgctgattgttcaaaactccttccctgtatcgcaggtcggtactgccacggcggctaataacttcttccgccagattggttcggcattgggtgcttccatcgtgggttcgatgttcattcacaatatgcagaatgagatggctacccgtttgcctgatgcccttgcatcgttgggcaaggaaggcgccgctatttcgcagcagttccaaggtgcagatgccgccaactccttgactccgcacgcagtcgcagagcttcccgatgtcctccgtgacgctatcttaaattcctacaatgacggtctgacccccgtgattggcatgatggtgccactggccattgttgcaatgctgattttgttcccactgcgccaagagcgcttgaaggaaaccatcgaataa

SEQ ID NO: 5 - DNA, 29 bp, Artificial Sequence
  impE1 kop-1
gctctagacgagaaagctaaagccggtga

SEQ ID NO: 6 - DNA, 36 bp, Artificial Sequence
  impE1 kop-2
gtttttagctaccattgttacaccccgtgcaagttt

SEQ ID NO: 7 - DNA, 36 bp, Artificial Sequence
  impE1 kop-3
gcacggggtgtaacaatggtagctaaaaactccacc

SEQ ID NO: 8 - DNA, 29 bp, Artificial Sequence
  impE1 kop-4
gctctagaaatagttggggaagtccactc

SEQ ID NO: 9 - DNA, 29 bp, Artificial Sequence
  impE2 kop-1
gctctagacttggatgacctggtggaaaa

SEQ ID NO: 10 - DNA, 36 bp, Artificial Sequence
  impE2 kop-2
cttggagaaaatttcctaccattccagtcctttcgt

SEQ ID NO: 11 - DNA, 36 bp, Artificial Sequence
  impE2 kop-3
ggactggaatggtaggaaattttctccaagggaaat

SEQ ID NO: 12 - DNA, 29 bp, Artificial Sequence
  impE2 kop-4
ggactagtggattgtgttgacgcacgatg

SEQ ID NO: 13 - DNA, 21 bp, Artificial Sequence
  impE1E2 seqF
gaacggagtcatctcctttgc

SEQ ID NO: 14 - DNA, 22 bp, Artificial Sequence
  impE1E2 seqR
ccaaacgctctgcaagaaactg

SEQ ID NO: 15 - DNA, 30 bp, Artificial Sequence
  XbaI-impE2 64 1F
gggtctagaaaagagcttaaggcagctgct

SEQ ID NO: 16 - DNA, 27 bp, Artificial Sequence
  impE2 64-R 1R
gaaaatcatctggcgcaaagagctcat

SEQ ID NO: 17 - DNA, 27 bp, Artificial Sequence
  impE2 64-H 1R
gaaaatcatctggtgcaaagagctcat

SEQ ID NO: 18 - DNA, 27 bp, Artificial Sequence
  impE2 64-D 1R
gaaaatcatctggtccaaagagctcat

SEQ ID NO: 19 - DNA, 27 bp, Artificial Sequence
  impE2 64-K 1R
gaaaatcatctgcttcaaagagctcat

SEQ ID NO: 20 - DNA, 27 bp, Artificial Sequence
  impE2 64-S 1R
gaaaatcatctgggacaaagagctcat

SEQ ID NO: 21 - DNA, 27 bp, Artificial Sequence
  impE2 64-T 1R
gaaaatcatctgggtcaaagagctcat

SEQ ID NO: 22 - DNA, 27 bp, Artificial Sequence
  impE2 64-N 1R
gaaaatcatctggttcaaagagctcat

SEQ ID NO: 23 - DNA, 27 bp, Artificial Sequence
  impE2 64-Q 1R
gaaaatcatctgctgcaaagagctcat

SEQ ID NO: 24 - DNA, 27 bp, Artificial Sequence
  impE2 64-C 1R
gaaaatcatctggcacaaagagctcat

SEQ ID NO: 25 - DNA, 27 bp, Artificial Sequence
  impE2 64-P 1R
gaaaatcatctgtggcaaagagctcat

SEQ ID NO: 26 - DNA, 27 bp, Artificial Sequence
  impE2 64-A 1R
gaaaatcatctgagccaaagagctcat

SEQ ID NO: 27 - DNA, 27 bp, Artificial Sequence
  impE2 64-V 1R
gaaaatcatctggaccaaagagctcat

SEQ ID NO: 28 - DNA, 27 bp, Artificial Sequence
  impE2 64-I 1R
gaaaatcatctggatcaaagagctcat

SEQ ID NO: 29 - DNA, 27 bp, Artificial Sequence
  impE2 64-L 1R
gaaaatcatctgcagcaaagagctcat

SEQ ID NO: 30 - DNA, 27 bp, Artificial Sequence
  impE2 64-M 1R
gaaaatcatctgcatcaaagagctcat

SEQ ID NO: 31 - DNA, 27 bp, Artificial Sequence
  impE2 64-F 1R
gaaaatcatctggaacaaagagctcat

SEQ ID NO: 32 - DNA, 27 bp, Artificial Sequence
  impE2 64-Y 1R
gaaaatcatctggtacaaagagctcat

SEQ ID NO: 33 - DNA, 27 bp, Artificial Sequence
  impE2 64-W 1R
gaaaatcatctgccacaaagagctcat

SEQ ID NO: 34 - DNA, 30 bp, Artificial Sequence
  XbaI-impE2 64 2R
gggtctagacggtcaatgaagtctcaacgg

SEQ ID NO: 35 - DNA, 27 bp, Artificial Sequence
  impE2 64-R 2F
atgagctctttgcgccagatgattttc

SEQ ID NO: 36 - DNA, 27 bp, Artificial Sequence
  impE2 64-H 2F
atgagctctttgcaccagatgattttc

SEQ ID NO: 37 - DNA, 27 bp, Artificial Sequence
  impE2 64-D 2F
atgagctctttggaccagatgattttc

SEQ ID NO: 38 - DNA, 27 bp, Artificial Sequence
  impE2 64-K 2F
atgagctctttgaagcagatgattttc

SEQ ID NO: 39 - DNA, 27 bp, Artificial Sequence
  impE2 64-S 2F
atgagctctttgtcccagatgattttc

SEQ ID NO: 40 - DNA, 27 bp, Artificial Sequence
  impE2 64-T 2F
atgagctctttgacccagatgattttc

SEQ ID NO: 41 - DNA, 27 bp, Artificial Sequence
  impE2 64-N 2F
atgagctctttgaaccagatgattttc

SEQ ID NO: 42 - DNA, 27 bp, Artificial Sequence
  impE2 64-Q 2F
atgagctctttgcagcagatgattttc

SEQ ID NO: 43 - DNA, 27 bp, Artificial Sequence
  impE2 64-C 2F
atgagctctttgtgccagatgattttc

SEQ ID NO: 44 - DNA, 27 bp, Artificial Sequence
  impE2 64-P 2F
atgagctctttgccacagatgattttc

SEQ ID NO: 45 - DNA, 27 bp, Artificial Sequence
  impE2 64-A 2F
atgagctctttggctcagatgattttc

SEQ ID NO: 46 - DNA, 27 bp, Artificial Sequence
  impE2 64-V 2F
atgagctctttggtccagatgattttc

SEQ ID NO: 47 - DNA, 27 bp, Artificial Sequence
  impE2 64-I 2F
atgagctctttgatccagatgattttc

SEQ ID NO: 48 - DNA, 27 bp, Artificial Sequence
  impE2 64-L 2F
atgagctctttgctgcagatgattttc

SEQ ID NO: 49 - DNA, 27 bp, Artificial Sequence
  impE2 64-M 2F
atgagctctttgatgcagatgattttc

SEQ ID NO: 50 - DNA, 27 bp, Artificial Sequence
  impE2 64-F 2F
atgagctctttgttccagatgattttc

SEQ ID NO: 51 - DNA, 27 bp, Artificial Sequence
  impE2 64-Y 2F
atgagctctttgtaccagatgattttc

SEQ ID NO: 52 - DNA, 27 bp, Artificial Sequence
  impE2 64-W 2F
atgagctctttgtggcagatgattttc

SEQ ID NO: 53 - DNA, 22 bp, Artificial Sequence
  impE lib F
cagatgattttcggttccgctc

SEQ ID NO: 54 - DNA, 23 bp, Artificial Sequence
  impE lib R
gaccgagacaaaaacgccaaacg

SEQ ID NO: 55 - DNA, 29 bp, Artificial Sequence
  impE mt - R
catctagaccgagacaaaaacgccaaacg

SEQ ID NO: 56 - DNA, 29 bp, Artificial Sequence
  impEW mt - 1
gctctagaccgcggataacgtcggcatta

SEQ ID NO: 57 - DNA, 21 bp, Artificial Sequence
  impEW ttk - 2
catccaccacaaagcaaacgc

SEQ ID NO: 58 - DNA, 36 bp, Artificial Sequence
  impEW ttk - 3
ctttgtggtggatgacccagatgaccgttgagactt

SEQ ID NO: 59 - DNA, 21 bp, Artificial Sequence
  impEW C - 2
aaatggagatacctgagatgt

SEQ ID NO: 60 - DNA, 36 bp, Artificial Sequence
  impEW C - 3
caggtatctccatttgcgttattggctcgacgctcg

SEQ ID NO: 61 - DNA, 21 bp, Artificial Sequence
  impEW v - 2
ggccgcaaaacccatccagtc

SEQ ID NO: 62 - DNA, 36 bp, Artificial Sequence
  impEW v - 3
atgggttttgcggccgtcgcaatcacgaccagcacc

SEQ ID NO: 63 - DNA, 21 bp, Artificial Sequence
  impEW y - 2
atacaaggaagcgaactccga

SEQ ID NO: 64 - DNA, 36 bp, Artificial Sequence
  impEW y - 3
ttcgcttccttgtatacggtgtcggcttgggctttg

SEQ ID NO: 65 - DNA, 36 bp, Artificial Sequence
  impE1E2 kop-2
cttggagaaaatttctgttacaccccgtgcaagttt

SEQ ID NO: 66 - DNA, 36 bp, Artificial Sequence
  impE1E2 kop-3
gcacggggtgtaacagaaattttctccaagggaaat

SEQ ID NO: 67 - DNA, 21 bp, Artificial Sequence
  impEW 387t - 2
catccaccacaaagcaaacgc

SEQ ID NO: 68 - DNA, 36 bp, Artificial Sequence; identical to SEQ ID NO: 58
  impEW 387t - 3

SEQ ID NO: 69 - DNA, 21 bp, Artificial Sequence
  impEW 413t - 2
tgacaaagcccaagccgacac

SEQ ID NO: 70 - DNA, 36 bp, Artificial Sequence
  impEW 413t - 3
cttgggctttgtcacgcaggtactggtgctgattgt

SEQ ID NO: 71 - DNA, 21 bp, Artificial Sequence
  impEW 458k- 2
ttgtgaatgaacatcgaaccc

SEQ ID NO: 72 - DNA, 36 bp, Artificial Sequence
  impEW 458k- 3
atgttcattcacaaaatgcagaatgagatggctacc

SEQ ID NO: 73 - protein, 549 aa, Unknown
  impE2(F123C)
MVAKNSTPSTAGHASAHTAEEFPVANAEMATPSAIDPNHGKKTADNVGIIFAALMLTMLMSSLGQMIFGSALPTIVGELGGVDQMSWVISAFMVTMTIAMPLAGQLGDRMGRKWVYISGISICVIGSTLGGFANGMGMLITGRAIQGFGAGIMMISSQSIVAEVVSARERGKFMGIMGGVFGVSSVLGPVLGGWFTDGPGWRWGLWINIPLGLLAIIVCAFVLKLRVGEQGFKGFDWMGFAAIAITTSTLILLTTWGGSEYEWTSPTILSMAAVVIVGALLTVFIESRASQPLIPVQLFKNRNMVLTTLAGTVLGLAMMGVLGYMPTYLQMVHTLTPTEAGLMMIPMMVGMIGVSTGVGFIIAKTGNYKYYPIAGLAITAFALWWMSQMTVETSLTGIGVRFLVFGVGLGFVMQVLVLIVQNSFPVSQVGTATAANNFFRQIGSALGASIVGSMFIHNMQNEMATRLPDALASLGKEGAAISQQFQGADAANSLTPHAVAELPDVLRDAILNSYNDGLTPVIGMMVPLAIVAMLILFPLRQERLKETIE

SEQ ID NO: 74 - protein, 549 aa, Unknown
  impE2(I243V)
MVAKNSTPSTAGHASAHTAEEFPVANAEMATPSAIDPNHGKKTADNVGIIFAALMLTMLMSSLGQMIFGSALPTIVGELGGVDQMSWVISAFMVTMTIAMPLAGQLGDRMGRKWVYISGISIFVIGSTLGGFANGMGMLITGRAIQGFGAGIMMISSQSIVAEVVSARERGKFMGIMGGVFGVSSVLGPVLGGWFTDGPGWRWGLWINIPLGLLAIIVCAFVLKLRVGEQGFKGFDWMGFAAVAITTSTLILLTTWGGSEYEWTSPTILSMAAVVIVGALLTVFIESRASQPLIPVQLFKNRNMVLTTLAGTVLGLAMMGVLGYMPTYLQMVHTLTPTEAGLMMIPMMVGMIGVSTGVGFIIAKTGNYKYYPIAGLAITAFALWWMSQMTVETSLTGIGVRFLVFGVGLGFVMQVLVLIVQNSFPVSQVGTATAANNFFRQIGSALGASIVGSMFIHNMQNEMATRLPDALASLGKEGAAISQQFQGADAANSLTPHAVAELPDVLRDAILNSYNDGLTPVIGMMVPLAIVAMLILFPLRQERLKETIE

SEQ ID NO: 75 - protein, 549 aa, Unknown
  impE2(S387T)
MVAKNSTPSTAGHASAHTAEEFPVANAEMATPSAIDPNHGKKTADNVGIIFAALMLTMLMSSLGQMIFGSALPTIVGELGGVDQMSWVISAFMVTMTIAMPLAGQLGDRMGRKWVYISGISIFVIGSTLGGFANGMGMLITGRAIQGFGAGIMMISSQSIVAEVVSARERGKFMGIMGGVFGVSSVLGPVLGGWFTDGPGWRWGLWINIPLGLLAIIVCAFVLKLRVGEQGFKGFDWMGFAAIAITTSTLILLTTWGGSEYEWTSPTILSMAAVVIVGALLTVFIESRASQPLIPVQLFKNRNMVLTTLAGTVLGLAMMGVLGYMPTYLQMVHTLTPTEAGLMMIPMMVGMIGVSTGVGFIIAKTGNYKYYPIAGLAITAFALWWMTQMTVETSLTGIGVRFLVFGVGLGFVMQVLVLIVQNSFPVSQVGTATAANNFFRQIGSALGASIVGSMFIHNMQNEMATRLPDALASLGKEGAAISQQFQGADAANSLTPHAVAELPDVLRDAILNSYNDGLTPVIGMMVPLAIVAMLILFPLRQERLKETIE

SEQ ID NO: 76 - protein, 549 aa, Unknown
  impE2(F405Y)
MVAKNSTPSTAGHASAHTAEEFPVANAEMATPSAIDPNHGKKTADNVGIIFAALMLTMLMSSLGQMIFGSALPTIVGELGGVDQMSWVISAFMVTMTIAMPLAGQLGDRMGRKWVYISGISIFVIGSTLGGFANGMGMLITGRAIQGFGAGIMMISSQSIVAEVVSARERGKFMGIMGGVFGVSSVLGPVLGGWFTDGPGWRWGLWINIPLGLLAIIVCAFVLKLRVGEQGFKGFDWMGFAAIAITTSTLILLTTWGGSEYEWTSPTILSMAAVVIVGALLTVFIESRASQPLIPVQLFKNRNMVLTTLAGTVLGLAMMGVLGYMPTYLQMVHTLTPTEAGLMMIPMMVGMIGVSTGVGFIIAKTGNYKYYPIAGLAITAFALWWMSQMTVETSLTGIGVRFLVYGVGLGFVMQVLVLIVQNSFPVSQVGTATAANNFFRQIGSALGASIVGSMFIHNMQNEMATRLPDALASLGKEGAAISQQFQGADAANSLTPHAVAELPDVLRDAILNSYNDGLTPVIGMMVPLAIVAMLILFPLRQERLKETIE

SEQ ID NO: 77 - protein, 549 aa, Unknown
  impE2(M413T)
MVAKNSTPSTAGHASAHTAEEFPVANAEMATPSAIDPNHGKKTADNVGIIFAALMLTMLMSSLGQMIFGSALPTIVGELGGVDQMSWVISAFMVTMTIAMPLAGQLGDRMGRKWVYISGISIFVIGSTLGGFANGMGMLITGRAIQGFGAGIMMISSQSIVAEVVSARERGKFMGIMGGVFGVSSVLGPVLGGWFTDGPGWRWGLWINIPLGLLAIIVCAFVLKLRVGEQGFKGFDWMGFAAIAITTSTLILLTTWGGSEYEWTSPTILSMAAVVIVGALLTVFIESRASQPLIPVQLFKNRNMVLTTLAGTVLGLAMMGVLGYMPTYLQMVHTLTPTEAGLMMIPMMVGMIGVSTGVGFIIAKTGNYKYYPIAGLAITAFALWWMSQMTVETSLTGIGVRFLVFGVGLGFVTQVLVLIVQNSFPVSQVGTATAANNFFRQIGSALGASIVGSMFIHNMQNEMATRLPDALASLGKEGAAISQQFQGADAANSLTPHAVAELPDVLRDAILNSYNDGLTPVIGMMVPLAIVAMLILFPLRQERLKETIE

SEQ ID NO: 78 - protein, 549 aa, Unknown
  impE2(N458K)
MVAKNSTPSTAGHASAHTAEEFPVANAEMATPSAIDPNHGKKTADNVGIIFAALMLTMLMSSLGQMIFGSALPTIVGELGGVDQMSWVISAFMVTMTIAMPLAGQLGDRMGRKWVYISGISIFVIGSTLGGFANGMGMLITGRAIQGFGAGIMMISSQSIVAEVVSARERGKFMGIMGGVFGVSSVLGPVLGGWFTDGPGWRWGLWINIPLGLLAIIVCAFVLKLRVGEQGFKGFDWMGFAAIAITTSTLILLTTWGGSEYEWTSPTILSMAAVVIVGALLTVFIESRASQPLIPVQLFKNRNMVLTTLAGTVLGLAMMGVLGYMPTYLQMVHTLTPTEAGLMMIPMMVGMIGVSTGVGFIIAKTGNYKYYPIAGLAITAFALWWMSQMTVETSLTGIGVRFLVFGVGLGFVMQVLVLIVQNSFPVSQVGTATAANNFFRQIGSALGASIVGSMFIHKMQNEMATRLPDALASLGKEGAAISQQFQGADAANSLTPHAVAELPDVLRDAILNSYNDGLTPVIGMMVPLAIVAMLILFPLRQERLKETIE

SEQ ID NO: 79 - DNA, 1650 bp, Unknown
  impE2(F123C)
atggtagctaaaaactccaccccaagcacggccggccacgccagtgctcacactgcggaagaattcccagtggccaatgctgaaatggcaacgccttcagcaatcgacccaaaccacggtaaaaagaccgcggataacgtcggcattatcttcgctgccttgatgctcaccatgctgatgagctctttggggcagatgattttcggttccgctctgccaaccatcgtcggcgagctcggcggcgtggaccagatgagctgggtaatttcagcatttatggtcaccatgaccattgctatgccactagccggtcagctcggtgaccgcatgggccgcaagtgggtctacatctcaggtatctccatttgcgttattggctcgacgctcggtggctttgccaatggcatgggcatgctgatcaccggacgtgcaatccagggcttcggtgccggcatcatgatgatttcctcgcagtcgattgtggctgaggttgtctccgcacgtgagcgcggcaagttcatgggtattatgggcggcgtctttggcgtctcctccgtactgggtccagttctcggtggctggttcaccgatggtcccggttggcgttggggcctgtggatcaacattccactgggtctgctggcaattattgtctgcgctttcgtactgaagctgcgcgtgggcgagcaaggctttaagggctttgactggatgggttttgcggccatcgcaatcacgaccagcaccctgattctgctcaccacttggggcggaagcgaatacgagtggacttccccaactattttgtccatggctgccgtagtcatcgtcggcgcgctgctcaccgtgttcattgagtcgcgtgcatcccagccgctgatcccggttcagctatttaagaaccgcaacatggttttgaccaccctcgccggtactgttttgggtctggccatgatgggcgtgctcggctacatgccaacctacctgcagatggtgcacaccctgacgccaactgaagcaggcttgatgatgatcccgatgatggtcggcatgatcggtgtctccactggtgttggcttcatcatcgctaagaccggcaactacaagtactaccccatcgcgggcctggccatcacggcgtttgctttgtggtggatgtcccagatgaccgttgagacttcattgaccggtatcggagttcgcttccttgtattcggtgtcggcttgggctttgtcatgcaggtactggtgctgattgttcaaaactccttccctgtatcgcaggtcggtactgccacggcggctaataacttcttccgccagattggttcggcattgggtgcttccatcgtgggttcgatgttcattcacaatatgcagaatgagatggctacccgtttgcctgatgcccttgcatcgttgggcaaggaaggcgccgctatttcgcagcagttccaaggtgcagatgccgccaactccttgactccgcacgcagtcgcagagcttcccgatgtcctccgtgacgctatcttaaattcctacaatgacggtctgacccccgtgattggcatgatggtgccactggccattgttgcaatgctgattttgttcccactgcgccaagagcgcttgaaggaaaccatcgaataa

SEQ ID NO: 80 - DNA, 1650 bp, Unknown
  impE2(I243V)
atggtagctaaaaactccaccccaagcacggccggccacgccagtgctcacactgcggaagaattcccagtggccaatgctgaaatggcaacgccttcagcaatcgacccaaaccacggtaaaaagaccgcggataacgtcggcattatcttcgctgccttgatgctcaccatgctgatgagctctttggggcagatgattttcggttccgctctgccaaccatcgtcggcgagctcggcggcgtggaccagatgagctgggtaatttcagcatttatggtcaccatgaccattgctatgccactagccggtcagctcggtgaccgcatgggccgcaagtgggtctacatctcaggtatctccattttcgttattggctcgacgctcggtggctttgccaatggcatgggcatgctgatcaccggacgtgcaatccagggcttcggtgccggcatcatgatgatttcctcgcagtcgattgtggctgaggttgtctccgcacgtgagcgcggcaagttcatgggtattatgggcggcgtctttggcgtctcctccgtactgggtccagttctcggtggctggttcaccgatggtcccggttggcgttggggcctgtggatcaacattccactgggtctgctggcaattattgtctgcgctttcgtactgaagctgcgcgtgggcgagcaaggctttaagggctttgactggatgggttttgcggccgtcgcaatcacgaccagcaccctgattctgctcaccacttggggcggaagcgaatacgagtggacttccccaactattttgtccatggctgccgtagtcatcgtcggcgcgctgctcaccgtgttcattgagtcgcgtgcatcccagccgctgatcccggttcagctatttaagaaccgcaacatggttttgaccaccctcgccggtactgttttgggtctggccatgatgggcgtgctcggctacatgccaacctacctgcagatggtgcacaccctgacgccaactgaagcaggcttgatgatgatcccgatgatggtcggcatgatcggtgtctccactggtgttggcttcatcatcgctaagaccggcaactacaagtactaccccatcgcgggcctggccatcacggcgtttgctttgtggtggatgtcccagatgaccgttgagacttcattgaccggtatcggagttcgcttccttgtattcggtgtcggcttgggctttgtcatgcaggtactggtgctgattgttcaaaactccttccctgtatcgcaggtcggtactgccacggcggctaataacttcttccgccagattggttcggcattgggtgcttccatcgtgggttcgatgttcattcacaatatgcagaatgagatggctacccgtttgcctgatgcccttgcatcgttgggcaaggaaggcgccgctatttcgcagcagttccaaggtgcagatgccgccaactccttgactccgcacgcagtcgcagagcttcccgatgtcctccgtgacgctatcttaaattcctacaatgacggtctgacccccgtgattggcatgatggtgccactggccattgttgcaatgctgattttgttcccactgcgccaagagcgcttgaaggaaaccatcgaataa

SEQ ID NO: 81 - DNA, 1650 bp, Unknown
  impE2(S387T)
atggtagctaaaaactccaccccaagcacggccggccacgccagtgctcacactgcggaagaattcccagtggccaatgctgaaatggcaacgccttcagcaatcgacccaaaccacggtaaaaagaccgcggataacgtcggcattatcttcgctgccttgatgctcaccatgctgatgagctctttggggcagatgattttcggttccgctctgccaaccatcgtcggcgagctcggcggcgtggaccagatgagctgggtaatttcagcatttatggtcaccatgaccattgctatgccactagccggtcagctcggtgaccgcatgggccgcaagtgggtctacatctcaggtatctccattttcgttattggctcgacgctcggtggctttgccaatggcatgggcatgctgatcaccggacgtgcaatccagggcttcggtgccggcatcatgatgatttcctcgcagtcgattgtggctgaggttgtctccgcacgtgagcgcggcaagttcatgggtattatgggcggcgtctttggcgtctcctccgtactgggtccagttctcggtggctggttcaccgatggtcccggttggcgttggggcctgtggatcaacattccactgggtctgctggcaattattgtctgcgctttcgtactgaagctgcgcgtgggcgagcaaggctttaagggctttgactggatgggttttgcggccatcgcaatcacgaccagcaccctgattctgctcaccacttggggcggaagcgaatacgagtggacttccccaactattttgtccatggctgccgtagtcatcgtcggcgcgctgctcaccgtgttcattgagtcgcgtgcatcccagccgctgatcccggttcagctatttaagaaccgcaacatggttttgaccaccctcgccggtactgttttgggtctggccatgatgggcgtgctcggctacatgccaacctacctgcagatggtgcacaccctgacgccaactgaagcaggcttgatgatgatcccgatgatggtcggcatgatcggtgtctccactggtgttggcttcatcatcgctaagaccggcaactacaagtactaccccatcgcgggcctggccatcacggcgtttgctttgtggtggatgacccagatgaccgttgagacttcattgaccggtatcggagttcgcttccttgtattcggtgtcggcttgggctttgtcatgcaggtactggtgctgattgttcaaaactccttccctgtatcgcaggtcggtactgccacggcggctaataacttcttccgccagattggttcggcattgggtgcttccatcgtgggttcgatgttcattcacaatatgcagaatgagatggctacccgtttgcctgatgcccttgcatcgttgggcaaggaaggcgccgctatttcgcagcagttccaaggtgcagatgccgccaactccttgactccgcacgcagtcgcagagcttcccgatgtcctccgtgacgctatcttaaattcctacaatgacggtctgacccccgtgattggcatgatggtgccactggccattgttgcaatgctgattttgttcccactgcgccaagagcgcttgaaggaaaccatcgaataa

SEQ ID NO: 82 - DNA, 1650 bp, Unknown
  impE2(F405Y)
atggtagctaaaaactccaccccaagcacggccggccacgccagtgctcacactgcggaagaattcccagtggccaatgctgaaatggcaacgccttcagcaatcgacccaaaccacggtaaaaagaccgcggataacgtcggcattatcttcgctgccttgatgctcaccatgctgatgagctctttggggcagatgattttcggttccgctctgccaaccatcgtcggcgagctcggcggcgtggaccagatgagctgggtaatttcagcatttatggtcaccatgaccattgctatgccactagccggtcagctcggtgaccgcatgggccgcaagtgggtctacatctcaggtatctccattttcgttattggctcgacgctcggtggctttgccaatggcatgggcatgctgatcaccggacgtgcaatccagggcttcggtgccggcatcatgatgatttcctcgcagtcgattgtggctgaggttgtctccgcacgtgagcgcggcaagttcatgggtattatgggcggcgtctttggcgtctcctccgtactgggtccagttctcggtggctggttcaccgatggtcccggttggcgttggggcctgtggatcaacattccactgggtctgctggcaattattgtctgcgctttcgtactgaagctgcgcgtgggcgagcaaggctttaagggctttgactggatgggttttgcggccatcgcaatcacgaccagcaccctgattctgctcaccacttggggcggaagcgaatacgagtggacttccccaactattttgtccatggctgccgtagtcatcgtcggcgcgctgctcaccgtgttcattgagtcgcgtgcatcccagccgctgatcccggttcagctatttaagaaccgcaacatggttttgaccaccctcgccggtactgttttgggtctggccatgatgggcgtgctcggctacatgccaacctacctgcagatggtgcacaccctgacgccaactgaagcaggcttgatgatgatcccgatgatggtcggcatgatcggtgtctccactggtgttggcttcatcatcgctaagaccggcaactacaagtactaccccatcgcgggcctggccatcacggcgtttgctttgtggtggatgtcccagatgaccgttgagacttcattgaccggtatcggagttcgcttccttgtatacggtgtcggcttgggctttgtcatgcaggtactggtgctgattgttcaaaactccttccctgtatcgcaggtcggtactgccacggcggctaataacttcttccgccagattggttcggcattgggtgcttccatcgtgggttcgatgttcattcacaatatgcagaatgagatggctacccgtttgcctgatgcccttgcatcgttgggcaaggaaggcgccgctatttcgcagcagttccaaggtgcagatgccgccaactccttgactccgcacgcagtcgcagagcttcccgatgtcctccgtgacgctatcttaaattcctacaatgacggtctgacccccgtgattggcatgatggtgccactggccattgttgcaatgctgattttgttcccactgcgccaagagcgcttgaaggaaaccatcgaataa

SEQ ID NO: 83 - DNA, 1650 bp, Unknown
  impE2(M413T)
atggtagctaaaaactccaccccaagcacggccggccacgccagtgctcacactgcggaagaattcccagtggccaatgctgaaatggcaacgccttcagcaatcgacccaaaccacggtaaaaagaccgcggataacgtcggcattatcttcgctgccttgatgctcaccatgctgatgagctctttggggcagatgattttcggttccgctctgccaaccatcgtcggcgagctcggcggcgtggaccagatgagctgggtaatttcagcatttatggtcaccatgaccattgctatgccactagccggtcagctcggtgaccgcatgggccgcaagtgggtctacatctcaggtatctccattttcgttattggctcgacgctcggtggctttgccaatggcatgggcatgctgatcaccggacgtgcaatccagggcttcggtgccggcatcatgatgatttcctcgcagtcgattgtggctgaggttgtctccgcacgtgagcgcggcaagttcatgggtattatgggcggcgtctttggcgtctcctccgtactgggtccagttctcggtggctggttcaccgatggtcccggttggcgttggggcctgtggatcaacattccactgggtctgctggcaattattgtctgcgctttcgtactgaagctgcgcgtgggcgagcaaggctttaagggctttgactggatgggttttgcggccatcgcaatcacgaccagcaccctgattctgctcaccacttggggcggaagcgaatacgagtggacttccccaactattttgtccatggctgccgtagtcatcgtcggcgcgctgctcaccgtgttcattgagtcgcgtgcatcccagccgctgatcccggttcagctatttaagaaccgcaacatggttttgaccaccctcgccggtactgttttgggtctggccatgatgggcgtgctcggctacatgccaacctacctgcagatggtgcacaccctgacgccaactgaagcaggcttgatgatgatcccgatgatggtcggcatgatcggtgtctccactggtgttggcttcatcatcgctaagaccggcaactacaagtactaccccatcgcgggcctggccatcacggcgtttgctttgtggtggatgtcccagatgaccgttgagacttcattgaccggtatcggagttcgcttccttgtattcggtgtcggcttgggctttgtcacgcaggtactggtgctgattgttcaaaactccttccctgtatcgcaggtcggtactgccacggcggctaataacttcttccgccagattggttcggcattgggtgcttccatcgtgggttcgatgttcattcacaatatgcagaatgagatggctacccgtttgcctgatgcccttgcatcgttgggcaaggaaggcgccgctatttcgcagcagttccaaggtgcagatgccgccaactccttgactccgcacgcagtcgcagagcttcccgatgtcctccgtgacgctatcttaaattcctacaatgacggtctgacccccgtgattggcatgatggtgccactggccattgttgcaatgctgattttgttcccactgcgccaagagcgcttgaaggaaaccatcgaataa

SEQ ID NO: 84 - DNA, 1650 bp, Unknown
  impE2(N458K)
atggtagctaaaaactccaccccaagcacggccggccacgccagtgctcacactgcggaagaattcccagtggccaatgctgaaatggcaacgccttcagcaatcgacccaaaccacggtaaaaagaccgcggataacgtcggcattatcttcgctgccttgatgctcaccatgctgatgagctctttggggcagatgattttcggttccgctctgccaaccatcgtcggcgagctcggcggcgtggaccagatgagctgggtaatttcagcatttatggtcaccatgaccattgctatgccactagccggtcagctcggtgaccgcatgggccgcaagtgggtctacatctcaggtatctccattttcgttattggctcgacgctcggtggctttgccaatggcatgggcatgctgatcaccggacgtgcaatccagggcttcggtgccggcatcatgatgatttcctcgcagtcgattgtggctgaggttgtctccgcacgtgagcgcggcaagttcatgggtattatgggcggcgtctttggcgtctcctccgtactgggtccagttctcggtggctggttcaccgatggtcccggttggcgttggggcctgtggatcaacattccactgggtctgctggcaattattgtctgcgctttcgtactgaagctgcgcgtgggcgagcaaggctttaagggctttgactggatgggttttgcggccatcgcaatcacgaccagcaccctgattctgctcaccacttggggcggaagcgaatacgagtggacttccccaactattttgtccatggctgccgtagtcatcgtcggcgcgctgctcaccgtgttcattgagtcgcgtgcatcccagccgctgatcccggttcagctatttaagaaccgcaacatggttttgaccaccctcgccggtactgttttgggtctggccatgatgggcgtgctcggctacatgccaacctacctgcagatggtgcacaccctgacgccaactgaagcaggcttgatgatgatcccgatgatggtcggcatgatcggtgtctccactggtgttggcttcatcatcgctaagaccggcaactacaagtactaccccatcgcgggcctggccatcacggcgtttgctttgtggtggatgtcccagatgaccgttgagacttcattgaccggtatcggagttcgcttccttgtattcggtgtcggcttgggctttgtcatgcaggtactggtgctgattgttcaaaactccttccctgtatcgcaggtcggtactgccacggcggctaataacttcttccgccagattggttcggcattgggtgcttccatcgtgggttcgatgttcattcacaaaatgcagaatgagatggctacccgtttgcctgatgcccttgcatcgttgggcaaggaaggcgccgctatttcgcagcagttccaaggtgcagatgccgccaactccttgactccgcacgcagtcgcagagcttcccgatgtcctccgtgacgctatcttaaattcctacaatgacggtctgacccccgtgattggcatgatggtgccactggccattgttgcaatgctgattttgttcccactgcgccaagagcgcttgaaggaaaccatcgaataa

SEQ ID NO: 85 - protein, 221 aa, Unknown
  ImpE1 - CJI0323
LHAVQEVNDNEEDSLPGSDLGLREQKRLATKHRIEDAATRLVDESSFDKVTIEEICEAAGISRRTFFNYFSTKESAVIGASSEPLTEKQRNDFLNADASNLLQLMVEQIKQHLESSHQSQAIHDRRQRIFADPDVAVRAMAFRKERSRETMELIAQRLREHPEKQRAPELDPETEAMLLSGFIREATWMAISRPDRDCALPVGDRIYRAMELVKNYTKGLE

SEQ ID NO: 86 - protein, 549 aa, Unknown
  ImpE2 - CJI0323
MIAKNSTPSTAGHASAHTAEEFPVANAEMATPSAIDPNHGKKTADNVGIIFAALMLTMLMSSLEQMIFGSALPTIVGELGGVDQMSWVISAFMVTMTIAMPLAGQLGDRMGRKWVYISGISIFVIGSTLGGFANGMGMLITGRAIQGFGAGIMMISSQSIVAEVVSARERGKFMGIMGGVFGVSSVLGPVLGGWFTDGPGWRWGLWINIPLGLLAIIVCAFVLKLRVGEQGFKGFDWMGFAAIAITTSTLILLTTWGGSEYEWTSPTILSMAAVVIVGALLTVFIESRASQPLIPVQLFKNRNMVLTTLAGTVLGLAMMGVLGYMPTYLQMVHTLTPTEAGLMMIPMMVGMIGVSTGVGFIIAKTGNYKYYPIAGLAITAFALWWMSQMTVETSLTGIGVRFLVFGVGLGFVMQVLVLIVQNSFPVSQVGTATAANNFFRQIGSALGASIVGSMFIHNMQNEMATRLPDALASLGKEGAAISQQFQGADAANSLTPHAVAELPDVLRDAILNSYNDGLTPVIGMMVPLAIVAMLILFPLRQERLKETIE

SEQ ID NO: 87 - DNA, 669 bp, Unknown
  ImpE1 NT - CJI0323
ttgcatgctgtgcaagaagttaatgacaatgaagaagactccctccctggcagtgacctcgggttaagggagcagaagcgattggcaaccaagcatcgcatcgaagacgccgcgacacggttggttgatgaatcgagctttgacaaagtaacaattgaagaaatttgcgaagccgccgggatttcccgacgcaccttttttaattatttcagcacgaaagaaagcgccgttattggcgcgtcctcggaaccgttgacggaaaagcaacgcaatgacttcttgaatgctgacgccagcaatctcctgcagctgatggttgagcagatcaaacaacacttggagtcttctcaccagagtcaagcgattcacgaccgtcgtcagcgaatctttgcggatccggatgtcgcggtacgtgcaatggcgtttcgcaaggaacgctcacgggaaaccatggagctaatcgctcaacgtcttcgggagcatcctgaaaaacaacgcgccccagaattggatccggaaacagaggcgatgctgctgagcggattcattcgcgaagccacctggatggctatctcacgacccgatcgtgattgtgcactgccagtgggtgaccgcatctatcgcgcgatggaattggtaaagaattacacgaaaggactggaatgatag

SEQ ID NO: 88 - DNA, 1650 bp, Unknown
  ImpE2 NT - CJI0323
atgatagctaaaaactccaccccaagcacggccggccacgccagtgctcacactgcggaagaattcccagtggccaatgctgaaatggcaacgccttcagcaatcgacccaaaccacggtaaaaagaccgcggataacgtcggcattatcttcgctgccttgatgctcaccatgctgatgagctctttggagcagatgattttcggttccgctctgccaaccatcgtcggcgagctcggcggcgtggaccagatgagctgggtaatttcagcatttatggtcaccatgaccattgctatgccactagccggtcagctcggtgaccgcatgggccgcaagtgggtctacatctcaggtatctccattttcgttattggctcgacgctcggtggctttgccaatggcatgggcatgctgatcaccggacgtgcaatccagggcttcggtgccggcatcatgatgatttcctcgcagtcgattgtggctgaggttgtctccgcacgtgagcgcggcaagttcatgggtattatgggcggcgtctttggcgtctcctccgtactgggtccagttctcggtggctggttcaccgatggtcccggttggcgttggggcctgtggatcaacattccactgggtctgctggcaattattgtctgcgctttcgtactgaagctgcgcgtgggcgagcaaggctttaagggctttgactggatgggttttgcggccatcgcaatcacgaccagcaccctgattctgctcaccacttggggcggaagcgaatacgagtggacttccccaactattttgtccatggctgccgtagtcatcgtcggcgcgctgctcaccgtgttcattgagtcgcgtgcatcccagccgctgatcccggttcagctatttaagaaccgcaacatggttttgaccaccctcgccggtactgttttgggtctggccatgatgggcgtgctcggctacatgccaacctacctgcagatggtgcacaccctgacgccaactgaagcaggcttgatgatgatcccgatgatggtcggcatgatcggtgtctccactggtgttggcttcatcatcgctaagaccggcaactacaagtactaccccatcgcgggcctggccatcacggcgtttgctttgtggtggatgtcccagatgaccgttgagacttcattgaccggtatcggagttcgcttccttgtattcggtgtcggcttgggctttgtcatgcaggtactggtgctgattgttcaaaactccttccctgtatcgcaggtcggtactgccacggcggctaataacttcttccgccagattggttcggcattgggtgcttccatcgtgggttcgatgttcattcacaatatgcagaatgagatggctacccgtttgcctgatgcccttgcatcgttgggcaaggaaggcgccgctatttcgcagcagttccaaggtgcagatgccgccaactccttgactccgcacgcagtcgcagagcttcccgatgtcctccgtgacgctatcttaaattcctacaatgacggtctgacccccgtgattggcatgatggtgccactggccattgttgcaatgctgattttgttcccactgcgccaagagcgcttgaaggaaaccatcgaataa

SEQ ID NO: 89 - DNA, 29 bp, Artificial Sequence
  impE1E2 WT F
gctctagagaacggagtcatctcctttgc

SEQ ID NO: 90 - DNA, 30 bp, Artificial Sequence
  impE1E2 WT R
gctctagaccaaacgctctgcaagaaactg

SEQ ID NO: 91 - DNA, 29 bp, Artificial Sequence
  impE1 164K-1
gctctagacttggatgacctggtggaaaa

SEQ ID NO: 92 - DNA, 37 bp, Artificial Sequence
  impE1 164K-2
ctggggcgcgttgtttttcaggatgctcccgaagacg

SEQ ID NO: 93 - DNA, 21 bp, Artificial Sequence
  impE1 164K-3
aacaacgcgccccagaattgg

SEQ ID NO: 94 - DNA, 29 bp, Artificial Sequence
  impE1 164K-4
gctctagaaatagttggggaagtccactc

SEQ ID NO: 95 - DNA, 37 bp, Artificial Sequence
  impE2 V2I-2
tggagtttttagctatcattccagtcctttcgtgtaa

SEQ ID NO: 96 - DNA, 21 bp, Artificial Sequence
  impE2 V2I-3
tagctaaaaactccaccccaa

SEQ ID NO: 97 - DNA, 37 bp, Artificial Sequence
  impE2 G64E-2
ccgaaaatcatctgctccaaagagctcatcagcatgg

SEQ ID NO: 98 - DNA, 21 bp, Artificial Sequence
  impE2 G64E-3
gcagatgattttcggttccgc

SEQ ID NO: 99 - protein, 549 aa, Unknown
  impE2 CJI0323 64D
MIAKNSTPSTAGHASAHTAEEFPVANAEMATPSAIDPNHGKKTADNVGIIFAALMLTMLMSSLDQMIFGSALPTIVGELGGVDQMSWVISAFMVTMTIAMPLAGQLGDRMGRKWVYISGISIFVIGSTLGGFANGMGMLITGRAIQGFGAGIMMISSQSIVAEVVSARERGKFMGIMGGVFGVSSVLGPVLGGWFTDGPGWRWGLWINIPLGLLAIIVCAFVLKLRVGEQGFKGFDWMGFAAIAITTSTLILLTTWGGSEYEWTSPTILSMAAVVIVGALLTVFIESRASQPLIPVQLFKNRNMVLTTLAGTVLGLAMMGVLGYMPTYLQMVHTLTPTEAGLMMIPMMVGMIGVSTGVGFIIAKTGNYKYYPIAGLAITAFALWWMSQMTVETSLTGIGVRFLVFGVGLGFVMQVLVLIVQNSFPVSQVGTATAANNFFRQIGSALGASIVGSMFIHNMQNEMATRLPDALASLGKEGAAISQQFQGADAANSLTPHAVAELPDVLRDAILNSYNDGLTPVIGMMVPLAIVAMLILFPLRQERLKETIE

SEQ ID NO: 100 - DNA, 1650 bp, Unknown
  impE2 CJI0323 64D
atgatagctaaaaactccaccccaagcacggccggccacgccagtgctcacactgcggaagaattcccagtggccaatgctgaaatggcaacgccttcagcaatcgacccaaaccacggtaaaaagaccgcggataacgtcggcattatcttcgctgccttgatgctcaccatgctgatgagctctttggaccagatgattttcggttccgctctgccaaccatcgtcggcgagctcggcggcgtggaccagatgagctgggtaatttcagcatttatggtcaccatgaccattgctatgccactagccggtcagctcggtgaccgcatgggccgcaagtgggtctacatctcaggtatctccattttcgttattggctcgacgctcggtggctttgccaatggcatgggcatgctgatcaccggacgtgcaatccagggcttcggtgccggcatcatgatgatttcctcgcagtcgattgtggctgaggttgtctccgcacgtgagcgcggcaagttcatgggtattatgggcggcgtctttggcgtctcctccgtactgggtccagttctcggtggctggttcaccgatggtcccggttggcgttggggcctgtggatcaacattccactgggtctgctggcaattattgtctgcgctttcgtactgaagctgcgcgtgggcgagcaaggctttaagggctttgactggatgggttttgcggccatcgcaatcacgaccagcaccctgattctgctcaccacttggggcggaagcgaatacgagtggacttccccaactattttgtccatggctgccgtagtcatcgtcggcgcgctgctcaccgtgttcattgagtcgcgtgcatcccagccgctgatcccggttcagctatttaagaaccgcaacatggttttgaccaccctcgccggtactgttttgggtctggccatgatgggcgtgctcggctacatgccaacctacctgcagatggtgcacaccctgacgccaactgaagcaggcttgatgatgatcccgatgatggtcggcatgatcggtgtctccactggtgttggcttcatcatcgctaagaccggcaactacaagtactaccccatcgcgggcctggccatcacggcgtttgctttgtggtggatgtcccagatgaccgttgagacttcattgaccggtatcggagttcgcttccttgtattcggtgtcggcttgggctttgtcatgcaggtactggtgctgattgttcaaaactccttccctgtatcgcaggtcggtactgccacggcggctaataacttcttccgccagattggttcggcattgggtgcttccatcgtgggttcgatgttcattcacaatatgcagaatgagatggctacccgtttgcctgatgcccttgcatcgttgggcaaggaaggcgccgctatttcgcagcagttccaaggtgcagatgccgccaactccttgactccgcacgcagtcgcagagcttcccgatgtcctccgtgacgctatcttaaattcctacaatgacggtctgacccccgtgattggcatgatggtgccactggccattgttgcaatgctgattttgttcccactgcgccaagagcgcttgaaggaaaccatcgaataa

SEQ ID NO: 101 - protein, 549 aa, Unknown
  impE2(S387T, M413T, N458K)
MVAKNSTPSTAGHASAHTAEEFPVANAEMATPSAIDPNHGKKTADNVGIIFAALMLTMLMSSLGQMIFGSALPTIVGELGGVDQMSWVISAFMVTMTIAMPLAGQLGDRMGRKWVYISGISIFVIGSTLGGFANGMGMLITGRAIQGFGAGIMMISSQSIVAEVVSARERGKFMGIMGGVFGVSSVLGPVLGGWFTDGPGWRWGLWINIPLGLLAIIVCAFVLKLRVGEQGFKGFDWMGFAAIAITTSTLILLTTWGGSEYEWTSPTILSMAAVVIVGALLTVFIESRASQPLIPVQLFKNRNMVLTTLAGTVLGLAMMGVLGYMPTYLQMVHTLTPTEAGLMMIPMMVGMIGVSTGVGFIIAKTGNYKYYPIAGLAITAFALWWMTQMTVETSLTGIGVRFLVFGVGLGFVTQVLVLIVQNSFPVSQVGTATAANNFFRQIGSALGASIVGSMFIHKMQNEMATRLPDALASLGKEGAAISQQFQGADAANSLTPHAVAELPDVLRDAILNSYNDGLTPVIGMMVPLAIVAMLILFPLRQERLKETIE

SEQ ID NO: 102 - DNA, 1650 bp, Unknown
  impE2(S387T, M413T, N458K)
atggtagctaaaaactccaccccaagcacggccggccacgccagtgctcacactgcggaagaattcccagtggccaatgctgaaatggcaacgccttcagcaatcgacccaaaccacggtaaaaagaccgcggataacgtcggcattatcttcgctgccttgatgctcaccatgctgatgagctctttggggcagatgattttcggttccgctctgccaaccatcgtcggcgagctcggcggcgtggaccagatgagctgggtaatttcagcatttatggtcaccatgaccattgctatgccactagccggtcagctcggtgaccgcatgggccgcaagtgggtctacatctcaggtatctccattttcgttattggctcgacgctcggtggctttgccaatggcatgggcatgctgatcaccggacgtgcaatccagggcttcggtgccggcatcatgatgatttcctcgcagtcgattgtggctgaggttgtctccgcacgtgagcgcggcaagttcatgggtattatgggcggcgtctttggcgtctcctccgtactgggtccagttctcggtggctggttcaccgatggtcccggttggcgttggggcctgtggatcaacattccactgggtctgctggcaattattgtctgcgctttcgtactgaagctgcgcgtgggcgagcaaggctttaagggctttgactggatgggttttgcggccatcgcaatcacgaccagcaccctgattctgctcaccacttggggcggaagcgaatacgagtggacttccccaactattttgtccatggctgccgtagtcatcgtcggcgcgctgctcaccgtgttcattgagtcgcgtgcatcccagccgctgatcccggttcagctatttaagaaccgcaacatggttttgaccaccctcgccggtactgttttgggtctggccatgatgggcgtgctcggctacatgccaacctacctgcagatggtgcacaccctgacgccaactgaagcaggcttgatgatgatcccgatgatggtcggcatgatcggtgtctccactggtgttggcttcatcatcgctaagaccggcaactacaagtactaccccatcgcgggcctggccatcacggcgtttgctttgtggtggatgacccagatgaccgttgagacttcattgaccggtatcggagttcgcttccttgtattcggtgtcggcttgggctttgtcacgcaggtactggtgctgattgttcaaaactccttccctgtatcgcaggtcggtactgccacggcggctaataacttcttccgccagattggttcggcattgggtgcttccatcgtgggttcgatgttcattcacaaaatgcagaatgagatggctacccgtttgcctgatgcccttgcatcgttgggcaaggaaggcgccgctatttcgcagcagttccaaggtgcagatgccgccaactccttgactccgcacgcagtcgcagagcttcccgatgtcctccgtgacgctatcttaaattcctacaatgacggtctgacccccgtgattggcatgatggtgccactggccattgttgcaatgctgattttgttcccactgcgccaagagcgcttgaaggaaaccatcgaataa

SEQ ID NO: 103 - protein, 549 aa, Unknown
  impE2(G64D, S387T, M413T, N458K)
MVAKNSTPSTAGHASAHTAEEFPVANAEMATPSAIDPNHGKKTADNVGIIFAALMLTMLMSSLDQMIFGSALPTIVGELGGVDQMSWVISAFMVTMTIAMPLAGQLGDRMGRKWVYISGISIFVIGSTLGGFANGMGMLITGRAIQGFGAGIMMISSQSIVAEVVSARERGKFMGIMGGVFGVSSVLGPVLGGWFTDGPGWRWGLWINIPLGLLAIIVCAFVLKLRVGEQGFKGFDWMGFAAIAITTSTLILLTTWGGSEYEWTSPTILSMAAVVIVGALLTVFIESRASQPLIPVQLFKNRNMVLTTLAGTVLGLAMMGVLGYMPTYLQMVHTLTPTEAGLMMIPMMVGMIGVSTGVGFIIAKTGNYKYYPIAGLAITAFALWWMTQMTVETSLTGIGVRFLVFGVGLGFVTQVLVLIVQNSFPVSQVGTATAANNFFRQIGSALGASIVGSMFIHKMQNEMATRLPDALASLGKEGAAISQQFQGADAANSLTPHAVAELPDVLRDAILNSYNDGLTPVIGMMVPLAIVAMLILFPLRQERLKETIE

SEQ ID NO: 104 - DNA, 1650 bp, Unknown
  impE2(G64D, S387T, M413T, N458K)
atggtagctaaaaactccaccccaagcacggccggccacgccagtgctcacactgcggaagaattcccagtggccaatgctgaaatggcaacgccttcagcaatcgacccaaaccacggtaaaaagaccgcggataacgtcggcattatcttcgctgccttgatgctcaccatgctgatgagctctttggaccagatgattttcggttccgctctgccaaccatcgtcggcgagctcggcggcgtggaccagatgagctgggtaatttcagcatttatggtcaccatgaccattgctatgccactagccggtcagctcggtgaccgcatgggccgcaagtgggtctacatctcaggtatctccattttcgttattggctcgacgctcggtggctttgccaatggcatgggcatgctgatcaccggacgtgcaatccagggcttcggtgccggcatcatgatgatttcctcgcagtcgattgtggctgaggttgtctccgcacgtgagcgcggcaagttcatgggtattatgggcggcgtctttggcgtctcctccgtactgggtccagttctcggtggctggttcaccgatggtcccggttggcgttggggcctgtggatcaacattccactgggtctgctggcaattattgtctgcgctttcgtactgaagctgcgcgtgggcgagcaaggctttaagggctttgactggatgggttttgcggccatcgcaatcacgaccagcaccctgattctgctcaccacttggggcggaagcgaatacgagtggacttccccaactattttgtccatggctgccgtagtcatcgtcggcgcgctgctcaccgtgttcattgagtcgcgtgcatcccagccgctgatcccggttcagctatttaagaaccgcaacatggttttgaccaccctcgccggtactgttttgggtctggccatgatgggcgtgctcggctacatgccaacctacctgcagatggtgcacaccctgacgccaactgaagcaggcttgatgatgatcccgatgatggtcggcatgatcggtgtctccactggtgttggcttcatcatcgctaagaccggcaactacaagtactaccccatcgcgggcctggccatcacggcgtttgctttgtggtggatgacccagatgaccgttgagacttcattgaccggtatcggagttcgcttccttgtattcggtgtcggcttgggctttgtcacgcaggtactggtgctgattgttcaaaactccttccctgtatcgcaggtcggtactgccacggcggctaataacttcttccgccagattggttcggcattgggtgcttccatcgtgggttcgatgttcattcacaaaatgcagaatgagatggctacccgtttgcctgatgcccttgcatcgttgggcaaggaaggcgccgctatttcgcagcagttccaaggtgcagatgccgccaactccttgactccgcacgcagtcgcagagcttcccgatgtcctccgtgacgctatcttaaattcctacaatgacggtctgacccccgtgattggcatgatggtgccactggccattgttgcaatgctgattttgttcccactgcgccaagagcgcttgaaggaaaccatcgaataa

SEQ ID NO: 105 - protein, 549 aa, Unknown
  impE2(G64D, F123C)
MVAKNSTPSTAGHASAHTAEEFPVANAEMATPSAIDPNHGKKTADNVGIIFAALMLTMLMSSLDQMIFGSALPTIVGELGGVDQMSWVISAFMVTMTIAMPLAGQLGDRMGRKWVYISGISICVIGSTLGGFANGMGMLITGRAIQGFGAGIMMISSQSIVAEVVSARERGKFMGIMGGVFGVSSVLGPVLGGWFTDGPGWRWGLWINIPLGLLAIIVCAFVLKLRVGEQGFKGFDWMGFAAIAITTSTLILLTTWGGSEYEWTSPTILSMAAVVIVGALLTVFIESRASQPLIPVQLFKNRNMVLTTLAGTVLGLAMMGVLGYMPTYLQMVHTLTPTEAGLMMIPMMVGMIGVSTGVGFIIAKTGNYKYYPIAGLAITAFALWWMSQMTVETSLTGIGVRFLVFGVGLGFVMQVLVLIVQNSFPVSQVGTATAANNFFRQIGSALGASIVGSMFIHNMQNEMATRLPDALASLGKEGAAISQQFQGADAANSLTPHAVAELPDVLRDAILNSYNDGLTPVIGMMVPLAIVAMLILFPLRQERLKETIE

SEQ ID NO: 106 - DNA, 1650 bp, Unknown
  impE2(G64D, F123C)
atggtagctaaaaactccaccccaagcacggccggccacgccagtgctcacactgcggaagaattcccagtggccaatgctgaaatggcaacgccttcagcaatcgacccaaaccacggtaaaaagaccgcggataacgtcggcattatcttcgctgccttgatgctcaccatgctgatgagctctttggaccagatgattttcggttccgctctgccaaccatcgtcggcgagctcggcggcgtggaccagatgagctgggtaatttcagcatttatggtcaccatgaccattgctatgccactagccggtcagctcggtgaccgcatgggccgcaagtgggtctacatctcaggtatctccatttgcgttattggctcgacgctcggtggctttgccaatggcatgggcatgctgatcaccggacgtgcaatccagggcttcggtgccggcatcatgatgatttcctcgcagtcgattgtggctgaggttgtctccgcacgtgagcgcggcaagttcatgggtattatgggcggcgtctttggcgtctcctccgtactgggtccagttctcggtggctggttcaccgatggtcccggttggcgttggggcctgtggatcaacattccactgggtctgctggcaattattgtctgcgctttcgtactgaagctgcgcgtgggcgagcaaggctttaagggctttgactggatgggttttgcggccatcgcaatcacgaccagcaccctgattctgctcaccacttggggcggaagcgaatacgagtggacttccccaactattttgtccatggctgccgtagtcatcgtcggcgcgctgctcaccgtgttcattgagtcgcgtgcatcccagccgctgatcccggttcagctatttaagaaccgcaacatggttttgaccaccctcgccggtactgttttgggtctggccatgatgggcgtgctcggctacatgccaacctacctgcagatggtgcacaccctgacgccaactgaagcaggcttgatgatgatcccgatgatggtcggcatgatcggtgtctccactggtgttggcttcatcatcgctaagaccggcaactacaagtactaccccatcgcgggcctggccatcacggcgtttgctttgtggtggatgtcccagatgaccgttgagacttcattgaccggtatcggagttcgcttccttgtattcggtgtcggcttgggctttgtcatgcaggtactggtgctgattgttcaaaactccttccctgtatcgcaggtcggtactgccacggcggctaataacttcttccgccagattggttcggcattgggtgcttccatcgtgggttcgatgttcattcacaatatgcagaatgagatggctacccgtttgcctgatgcccttgcatcgttgggcaaggaaggcgccgctatttcgcagcagttccaaggtgcagatgccgccaactccttgactccgcacgcagtcgcagagcttcccgatgtcctccgtgacgctatcttaaattcctacaatgacggtctgacccccgtgattggcatgatggtgccactggccattgttgcaatgctgattttgttcccactgcgccaagagcgcttgaaggaaaccatcgaataa

SEQ ID NO: 107 - protein, 549 aa, Unknown
  impE2(G64D, I243V)
MVAKNSTPSTAGHASAHTAEEFPVANAEMATPSAIDPNHGKKTADNVGIIFAALMLTMLMSSLDQMIFGSALPTIVGELGGVDQMSWVISAFMVTMTIAMPLAGQLGDRMGRKWVYISGISIFVIGSTLGGFANGMGMLITGRAIQGFGAGIMMISSQSIVAEVVSARERGKFMGIMGGVFGVSSVLGPVLGGWFTDGPGWRWGLWINIPLGLLAIIVCAFVLKLRVGEQGFKGFDWMGFAAVAITTSTLILLTTWGGSEYEWTSPTILSMAAVVIVGALLTVFIESRASQPLIPVQLFKNRNMVLTTLAGTVLGLAMMGVLGYMPTYLQMVHTLTPTEAGLMMIPMMVGMIGVSTGVGFIIAKTGNYKYYPIAGLAITAFALWWMSQMTVETSLTGIGVRFLVFGVGLGFVMQVLVLIVQNSFPVSQVGTATAANNFFRQIGSALGASIVGSMFIHNMQNEMATRLPDALASLGKEGAAISQQFQGADAANSLTPHAVAELPDVLRDAILNSYNDGLTPVIGMMVPLAIVAMLILFPLRQERLKETIE

SEQ ID NO: 108 - DNA, 1650 bp, Unknown
  impE2(G64D, I243V)
atggtagctaaaaactccaccccaagcacggccggccacgccagtgctcacactgcggaagaattcccagtggccaatgctgaaatggcaacgccttcagcaatcgacccaaaccacggtaaaaagaccgcggataacgtcggcattatcttcgctgccttgatgctcaccatgctgatgagctctttggaccagatgattttcggttccgctctgccaaccatcgtcggcgagctcggcggcgtggaccagatgagctgggtaatttcagcatttatggtcaccatgaccattgctatgccactagccggtcagctcggtgaccgcatgggccgcaagtgggtctacatctcaggtatctccattttcgttattggctcgacgctcggtggctttgccaatggcatgggcatgctgatcaccggacgtgcaatccagggcttcggtgccggcatcatgatgatttcctcgcagtcgattgtggctgaggttgtctccgcacgtgagcgcggcaagttcatgggtattatgggcggcgtctttggcgtctcctccgtactgggtccagttctcggtggctggttcaccgatggtcccggttggcgttggggcctgtggatcaacattccactgggtctgctggcaattattgtctgcgctttcgtactgaagctgcgcgtgggcgagcaaggctttaagggctttgactggatgggttttgcggccgtcgcaatcacgaccagcaccctgattctgctcaccacttggggcggaagcgaatacgagtggacttccccaactattttgtccatggctgccgtagtcatcgtcggcgcgctgctcaccgtgttcattgagtcgcgtgcatcccagccgctgatcccggttcagctatttaagaaccgcaacatggttttgaccaccctcgccggtactgttttgggtctggccatgatgggcgtgctcggctacatgccaacctacctgcagatggtgcacaccctgacgccaactgaagcaggcttgatgatgatcccgatgatggtcggcatgatcggtgtctccactggtgttggcttcatcatcgctaagaccggcaactacaagtactaccccatcgcgggcctggccatcacggcgtttgctttgtggtggatgtcccagatgaccgttgagacttcattgaccggtatcggagttcgcttccttgtattcggtgtcggcttgggctttgtcatgcaggtactggtgctgattgttcaaaactccttccctgtatcgcaggtcggtactgccacggcggctaataacttcttccgccagattggttcggcattgggtgcttccatcgtgggttcgatgttcattcacaatatgcagaatgagatggctacccgtttgcctgatgcccttgcatcgttgggcaaggaaggcgccgctatttcgcagcagttccaaggtgcagatgccgccaactccttgactccgcacgcagtcgcagagcttcccgatgtcctccgtgacgctatcttaaattcctacaatgacggtctgacccccgtgattggcatgatggtgccactggccattgttgcaatgctgattttgttcccactgcgccaagagcgcttgaaggaaaccatcgaataa

SEQ ID NO: 109 - protein, 549 aa, Unknown
  impE2(G64D, F405Y)
MVAKNSTPSTAGHASAHTAEEFPVANAEMATPSAIDPNHGKKTADNVGIIFAALMLTMLMSSLDQMIFGSALPTIVGELGGVDQMSWVISAFMVTMTIAMPLAGQLGDRMGRKWVYISGISIFVIGSTLGGFANGMGMLITGRAIQGFGAGIMMISSQSIVAEVVSARERGKFMGIMGGVFGVSSVLGPVLGGWFTDGPGWRWGLWINIPLGLLAIIVCAFVLKLRVGEQGFKGFDWMGFAAIAITTSTLILLTTWGGSEYEWTSPTILSMAAVVIVGALLTVFIESRASQPLIPVQLFKNRNMVLTTLAGTVLGLAMMGVLGYMPTYLQMVHTLTPTEAGLMMIPMMVGMIGVSTGVGFIIAKTGNYKYYPIAGLAITAFALWWMSQMTVETSLTGIGVRFLVYGVGLGFVMQVLVLIVQNSFPVSQVGTATAANNFFRQIGSALGASIVGSMFIHNMQNEMATRLPDALASLGKEGAAISQQFQGADAANSLTPHAVAELPDVLRDAILNSYNDGLTPVIGMMVPLAIVAMLILFPLRQERLKETIE

SEQ ID NO: 110 - DNA, 1650 bp, Unknown
  impE2(G64D, F405Y)
atggtagctaaaaactccaccccaagcacggccggccacgccagtgctcacactgcggaagaattcccagtggccaatgctgaaatggcaacgccttcagcaatcgacccaaaccacggtaaaaagaccgcggataacgtcggcattatcttcgctgccttgatgctcaccatgctgatgagctctttggaccagatgattttcggttccgctctgccaaccatcgtcggcgagctcggcggcgtggaccagatgagctgggtaatttcagcatttatggtcaccatgaccattgctatgccactagccggtcagctcggtgaccgcatgggccgcaagtgggtctacatctcaggtatctccattttcgttattggctcgacgctcggtggctttgccaatggcatgggcatgctgatcaccggacgtgcaatccagggcttcggtgccggcatcatgatgatttcctcgcagtcgattgtggctgaggttgtctccgcacgtgagcgcggcaagttcatgggtattatgggcggcgtctttggcgtctcctccgtactgggtccagttctcggtggctggttcaccgatggtcccggttggcgttggggcctgtggatcaacattccactgggtctgctggcaattattgtctgcgctttcgtactgaagctgcgcgtgggcgagcaaggctttaagggctttgactggatgggttttgcggccatcgcaatcacgaccagcaccctgattctgctcaccacttggggcggaagcgaatacgagtggacttccccaactattttgtccatggctgccgtagtcatcgtcggcgcgctgctcaccgtgttcattgagtcgcgtgcatcccagccgctgatcccggttcagctatttaagaaccgcaacatggttttgaccaccctcgccggtactgttttgggtctggccatgatgggcgtgctcggctacatgccaacctacctgcagatggtgcacaccctgacgccaactgaagcaggcttgatgatgatcccgatgatggtcggcatgatcggtgtctccactggtgttggcttcatcatcgctaagaccggcaactacaagtactaccccatcgcgggcctggccatcacggcgtttgctttgtggtggatgtcccagatgaccgttgagacttcattgaccggtatcggagttcgcttccttgtatacggtgtcggcttgggctttgtcatgcaggtactggtgctgattgttcaaaactccttccctgtatcgcaggtcggtactgccacggcggctaataacttcttccgccagattggttcggcattgggtgcttccatcgtgggttcgatgttcattcacaatatgcagaatgagatggctacccgtttgcctgatgcccttgcatcgttgggcaaggaaggcgccgctatttcgcagcagttccaaggtgcagatgccgccaactccttgactccgcacgcagtcgcagagcttcccgatgtcctccgtgacgctatcttaaattcctacaatgacggtctgacccccgtgattggcatgatggtgccactggccattgttgcaatgctgattttgttcccactgcgccaagagcgcttgaaggaaaccatcgaataa

SEQ ID NO: 111 - protein, 549 aa, Unknown
  impE2(F123C, I243V, S387T, F405Y, M413T, N458K)
MVAKNSTPSTAGHASAHTAEEFPVANAEMATPSAIDPNHGKKTADNVGIIFAALMLTMLMSSLGQMIFGSALPTIVGELGGVDQMSWVISAFMVTMTIAMPLAGQLGDRMGRKWVYISGISICVIGSTLGGFANGMGMLITGRAIQGFGAGIMMISSQSIVAEVVSARERGKFMGIMGGVFGVSSVLGPVLGGWFTDGPGWRWGLWINIPLGLLAIIVCAFVLKLRVGEQGFKGFDWMGFAAVAITTSTLILLTTWGGSEYEWTSPTILSMAAVVIVGALLTVFIESRASQPLIPVQLFKNRNMVLTTLAGTVLGLAMMGVLGYMPTYLQMVHTLTPTEAGLMMIPMMVGMIGVSTGVGFIIAKTGNYKYYPIAGLAITAFALWWMTQMTVETSLTGIGVRFLVYGVGLGFVTQVLVLIVQNSFPVSQVGTATAANNFFRQIGSALGASIVGSMFIHKMQNEMATRLPDALASLGKEGAAISQQFQGADAANSLTPHAVAELPDVLRDAILNSYNDGLTPVIGMMVPLAIVAMLILFPLRQERLKETIE

SEQ ID NO: 112 - DNA, 1650 bp, Unknown
  impE2(F123C, I243V, S387T, F405Y, M413T, N458K)
atggtagctaaaaactccaccccaagcacggccggccacgccagtgctcacactgcggaagaattcccagtggccaatgctgaaatggcaacgccttcagcaatcgacccaaaccacggtaaaaagaccgcggataacgtcggcattatcttcgctgccttgatgctcaccatgctgatgagctctttggggcagatgattttcggttccgctctgccaaccatcgtcggcgagctcggcggcgtggaccagatgagctgggtaatttcagcatttatggtcaccatgaccattgctatgccactagccggtcagctcggtgaccgcatgggccgcaagtgggtctacatctcaggtatctccatttgcgttattggctcgacgctcggtggctttgccaatggcatgggcatgctgatcaccggacgtgcaatccagggcttcggtgccggcatcatgatgatttcctcgcagtcgattgtggctgaggttgtctccgcacgtgagcgcggcaagttcatgggtattatgggcggcgtctttggcgtctcctccgtactgggtccagttctcggtggctggttcaccgatggtcccggttggcgttggggcctgtggatcaacattccactgggtctgctggcaattattgtctgcgctttcgtactgaagctgcgcgtgggcgagcaaggctttaagggctttgactggatgggttttgcggccgtcgcaatcacgaccagcaccctgattctgctcaccacttggggcggaagcgaatacgagtggacttccccaactattttgtccatggctgccgtagtcatcgtcggcgcgctgctcaccgtgttcattgagtcgcgtgcatcccagccgctgatcccggttcagctatttaagaaccgcaacatggttttgaccaccctcgccggtactgttttgggtctggccatgatgggcgtgctcggctacatgccaacctacctgcagatggtgcacaccctgacgccaactgaagcaggcttgatgatgatcccgatgatggtcggcatgatcggtgtctccactggtgttggcttcatcatcgctaagaccggcaactacaagtactaccccatcgcgggcctggccatcacggcgtttgctttgtggtggatgacccagatgaccgttgagacttcattgaccggtatcggagttcgcttccttgtatacggtgtcggcttgggctttgtcacgcaggtactggtgctgattgttcaaaactccttccctgtatcgcaggtcggtactgccacggcggctaataacttcttccgccagattggttcggcattgggtgcttccatcgtgggttcgatgttcattcacaaaatgcagaatgagatggctacccgtttgcctgatgcccttgcatcgttgggcaaggaaggcgccgctatttcgcagcagttccaaggtgcagatgccgccaactccttgactccgcacgcagtcgcagagcttcccgatgtcctccgtgacgctatcttaaattcctacaatgacggtctgacccccgtgattggcatgatggtgccactggccattgttgcaatgctgattttgttcccactgcgccaagagcgcttgaaggaaaccatcgaataa

SEQ ID NO: 113 - protein, 549 aa, Unknown
  impE2(G64D, S387T)
MVAKNSTPSTAGHASAHTAEEFPVANAEMATPSAIDPNHGKKTADNVGIIFAALMLTMLMSSLDQMIFGSALPTIVGELGGVDQMSWVISAFMVTMTIAMPLAGQLGDRMGRKWVYISGISIFVIGSTLGGFANGMGMLITGRAIQGFGAGIMMISSQSIVAEVVSARERGKFMGIMGGVFGVSSVLGPVLGGWFTDGPGWRWGLWINIPLGLLAIIVCAFVLKLRVGEQGFKGFDWMGFAAIAITTSTLILLTTWGGSEYEWTSPTILSMAAVVIVGALLTVFIESRASQPLIPVQLFKNRNMVLTTLAGTVLGLAMMGVLGYMPTYLQMVHTLTPTEAGLMMIPMMVGMIGVSTGVGFIIAKTGNYKYYPIAGLAITAFALWWMTQMTVETSLTGIGVRFLVFGVGLGFVMQVLVLIVQNSFPVSQVGTATAANNFFRQIGSALGASIVGSMFIHNMQNEMATRLPDALASLGKEGAAISQQFQGADAANSLTPHAVAELPDVLRDAILNSYNDGLTPVIGMMVPLAIVAMLILFPLRQERLKETIE

SEQ ID NO: 114 - DNA, 1650 bp, Unknown
  impE2(G64D, S387T)
atggtagctaaaaactccaccccaagcacggccggccacgccagtgctcacactgcggaagaattcccagtggccaatgctgaaatggcaacgccttcagcaatcgacccaaaccacggtaaaaagaccgcggataacgtcggcattatcttcgctgccttgatgctcaccatgctgatgagctctttggaccagatgattttcggttccgctctgccaaccatcgtcggcgagctcggcggcgtggaccagatgagctgggtaatttcagcatttatggtcaccatgaccattgctatgccactagccggtcagctcggtgaccgcatgggccgcaagtgggtctacatctcaggtatctccattttcgttattggctcgacgctcggtggctttgccaatggcatgggcatgctgatcaccggacgtgcaatccagggcttcggtgccggcatcatgatgatttcctcgcagtcgattgtggctgaggttgtctccgcacgtgagcgcggcaagttcatgggtattatgggcggcgtctttggcgtctcctccgtactgggtccagttctcggtggctggttcaccgatggtcccggttggcgttggggcctgtggatcaacattccactgggtctgctggcaattattgtctgcgctttcgtactgaagctgcgcgtgggcgagcaaggctttaagggctttgactggatgggttttgcggccatcgcaatcacgaccagcaccctgattctgctcaccacttggggcggaagcgaatacgagtggacttccccaactattttgtccatggctgccgtagtcatcgtcggcgcgctgctcaccgtgttcattgagtcgcgtgcatcccagccgctgatcccggttcagctatttaagaaccgcaacatggttttgaccaccctcgccggtactgttttgggtctggccatgatgggcgtgctcggctacatgccaacctacctgcagatggtgcacaccctgacgccaactgaagcaggcttgatgatgatcccgatgatggtcggcatgatcggtgtctccactggtgttggcttcatcatcgctaagaccggcaactacaagtactaccccatcgcgggcctggccatcacggcgtttgctttgtggtggatgacccagatgaccgttgagacttcattgaccggtatcggagttcgcttccttgtattcggtgtcggcttgggctttgtcatgcaggtactggtgctgattgttcaaaactccttccctgtatcgcaggtcggtactgccacggcggctaataacttcttccgccagattggttcggcattgggtgcttccatcgtgggttcgatgttcattcacaatatgcagaatgagatggctacccgtttgcctgatgcccttgcatcgttgggcaaggaaggcgccgctatttcgcagcagttccaaggtgcagatgccgccaactccttgactccgcacgcagtcgcagagcttcccgatgtcctccgtgacgctatcttaaattcctacaatgacggtctgacccccgtgattggcatgatggtgccactggccattgttgcaatgctgattttgttcccactgcgccaagagcgcttgaaggaaaccatcgaataa

SEQ ID NO: 115 - protein, 549 aa, Unknown
  impE2(G64D, M413T)
MVAKNSTPSTAGHASAHTAEEFPVANAEMATPSAIDPNHGKKTADNVGIIFAALMLTMLMSSLDQMIFGSALPTIVGELGGVDQMSWVISAFMVTMTIAMPLAGQLGDRMGRKWVYISGISIFVIGSTLGGFANGMGMLITGRAIQGFGAGIMMISSQSIVAEVVSARERGKFMGIMGGVFGVSSVLGPVLGGWFTDGPGWRWGLWINIPLGLLAIIVCAFVLKLRVGEQGFKGFDWMGFAAIAITTSTLILLTTWGGSEYEWTSPTILSMAAVVIVGALLTVFIESRASQPLIPVQLFKNRNMVLTTLAGTVLGLAMMGVLGYMPTYLQMVHTLTPTEAGLMMIPMMVGMIGVSTGVGFIIAKTGNYKYYPIAGLAITAFALWWMSQMTVETSLTGIGVRFLVFGVGLGFVTQVLVLIVQNSFPVSQVGTATAANNFFRQIGSALGASIVGSMFIHNMQNEMATRLPDALASLGKEGAAISQQFQGADAANSLTPHAVAELPDVLRDAILNSYNDGLTPVIGMMVPLAIVAMLILFPLRQERLKETIE

SEQ ID NO: 116 - DNA, 1650 bp, Unknown
  impE2(G64D, M413T)
atggtagctaaaaactccaccccaagcacggccggccacgccagtgctcacactgcggaagaattcccagtggccaatgctgaaatggcaacgccttcagcaatcgacccaaaccacggtaaaaagaccgcggataacgtcggcattatcttcgctgccttgatgctcaccatgctgatgagctctttggaccagatgattttcggttccgctctgccaaccatcgtcggcgagctcggcggcgtggaccagatgagctgggtaatttcagcatttatggtcaccatgaccattgctatgccactagccggtcagctcggtgaccgcatgggccgcaagtgggtctacatctcaggtatctccattttcgttattggctcgacgctcggtggctttgccaatggcatgggcatgctgatcaccggacgtgcaatccagggcttcggtgccggcatcatgatgatttcctcgcagtcgattgtggctgaggttgtctccgcacgtgagcgcggcaagttcatgggtattatgggcggcgtctttggcgtctcctccgtactgggtccagttctcggtggctggttcaccgatggtcccggttggcgttggggcctgtggatcaacattccactgggtctgctggcaattattgtctgcgctttcgtactgaagctgcgcgtgggcgagcaaggctttaagggctttgactggatgggttttgcggccatcgcaatcacgaccagcaccctgattctgctcaccacttggggcggaagcgaatacgagtggacttccccaactattttgtccatggctgccgtagtcatcgtcggcgcgctgctcaccgtgttcattgagtcgcgtgcatcccagccgctgatcccggttcagctatttaagaaccgcaacatggttttgaccaccctcgccggtactgttttgggtctggccatgatgggcgtgctcggctacatgccaacctacctgcagatggtgcacaccctgacgccaactgaagcaggcttgatgatgatcccgatgatggtcggcatgatcggtgtctccactggtgttggcttcatcatcgctaagaccggcaactacaagtactaccccatcgcgggcctggccatcacggcgtttgctttgtggtggatgtcccagatgaccgttgagacttcattgaccggtatcggagttcgcttccttgtattcggtgtcggcttgggctttgtcacgcaggtactggtgctgattgttcaaaactccttccctgtatcgcaggtcggtactgccacggcggctaataacttcttccgccagattggttcggcattgggtgcttccatcgtgggttcgatgttcattcacaatatgcagaatgagatggctacccgtttgcctgatgcccttgcatcgttgggcaaggaaggcgccgctatttcgcagcagttccaaggtgcagatgccgccaactccttgactccgcacgcagtcgcagagcttcccgatgtcctccgtgacgctatcttaaattcctacaatgacggtctgacccccgtgattggcatgatggtgccactggccattgttgcaatgctgattttgttcccactgcgccaagagcgcttgaaggaaaccatcgaataa

SEQ ID NO: 117 - protein, 549 aa, Unknown
  impE2(G64D, N458K)
MVAKNSTPSTAGHASAHTAEEFPVANAEMATPSAIDPNHGKKTADNVGIIFAALMLTMLMSSLDQMIFGSALPTIVGELGGVDQMSWVISAFMVTMTIAMPLAGQLGDRMGRKWVYISGISIFVIGSTLGGFANGMGMLITGRAIQGFGAGIMMISSQSIVAEVVSARERGKFMGIMGGVFGVSSVLGPVLGGWFTDGPGWRWGLWINIPLGLLAIIVCAFVLKLRVGEQGFKGFDWMGFAAIAITTSTLILLTTWGGSEYEWTSPTILSMAAVVIVGALLTVFIESRASQPLIPVQLFKNRNMVLTTLAGTVLGLAMMGVLGYMPTYLQMVHTLTPTEAGLMMIPMMVGMIGVSTGVGFIIAKTGNYKYYPIAGLAITAFALWWMSQMTVETSLTGIGVRFLVFGVGLGFVMQVLVLIVQNSFPVSQVGTATAANNFFRQIGSALGASIVGSMFIHKMQNEMATRLPDALASLGKEGAAISQQFQGADAANSLTPHAVAELPDVLRDAILNSYNDGLTPVIGMMVPLAIVAMLILFPLRQERLKETIE

SEQ ID NO: 118 - DNA, 1650 bp, Unknown
  impE2(G64D, N458K)
atggtagctaaaaactccaccccaagcacggccggccacgccagtgctcacactgcggaagaattcccagtggccaatgctgaaatggcaacgccttcagcaatcgacccaaaccacggtaaaaagaccgcggataacgtcggcattatcttcgctgccttgatgctcaccatgctgatgagctctttggaccagatgattttcggttccgctctgccaaccatcgtcggcgagctcggcggcgtggaccagatgagctgggtaatttcagcatttatggtcaccatgaccattgctatgccactagccggtcagctcggtgaccgcatgggccgcaagtgggtctacatctcaggtatctccattttcgttattggctcgacgctcggtggctttgccaatggcatgggcatgctgatcaccggacgtgcaatccagggcttcggtgccggcatcatgatgatttcctcgcagtcgattgtggctgaggttgtctccgcacgtgagcgcggcaagttcatgggtattatgggcggcgtctttggcgtctcctccgtactgggtccagttctcggtggctggttcaccgatggtcccggttggcgttggggcctgtggatcaacattccactgggtctgctggcaattattgtctgcgctttcgtactgaagctgcgcgtgggcgagcaaggctttaagggctttgactggatgggttttgcggccatcgcaatcacgaccagcaccctgattctgctcaccacttggggcggaagcgaatacgagtggacttccccaactattttgtccatggctgccgtagtcatcgtcggcgcgctgctcaccgtgttcattgagtcgcgtgcatcccagccgctgatcccggttcagctatttaagaaccgcaacatggttttgaccaccctcgccggtactgttttgggtctggccatgatgggcgtgctcggctacatgccaacctacctgcagatggtgcacaccctgacgccaactgaagcaggcttgatgatgatcccgatgatggtcggcatgatcggtgtctccactggtgttggcttcatcatcgctaagaccggcaactacaagtactaccccatcgcgggcctggccatcacggcgtttgctttgtggtggatgtcccagatgaccgttgagacttcattgaccggtatcggagttcgcttccttgtattcggtgtcggcttgggctttgtcatgcaggtactggtgctgattgttcaaaactccttccctgtatcgcaggtcggtactgccacggcggctaataacttcttccgccagattggttcggcattgggtgcttccatcgtgggttcgatgttcattcacaaaatgcagaatgagatggctacccgtttgcctgatgcccttgcatcgttgggcaaggaaggcgccgctatttcgcagcagttccaaggtgcagatgccgccaactccttgactccgcacgcagtcgcagagcttcccgatgtcctccgtgacgctatcttaaattcctacaatgacggtctgacccccgtgattggcatgatggtgccactggccattgttgcaatgctgattttgttcccactgcgccaagagcgcttgaaggaaaccatcgaataa

SEQ ID NO: 119 - protein, 549 aa, Unknown
  impE2(G64D, I243V, S387T, M413T, N458K)
MVAKNSTPSTAGHASAHTAEEFPVANAEMATPSAIDPNHGKKTADNVGIIFAALMLTMLMSSLDQMIFGSALPTIVGELGGVDQMSWVISAFMVTMTIAMPLAGQLGDRMGRKWVYISGISIFVIGSTLGGFANGMGMLITGRAIQGFGAGIMMISSQSIVAEVVSARERGKFMGIMGGVFGVSSVLGPVLGGWFTDGPGWRWGLWINIPLGLLAIIVCAFVLKLRVGEQGFKGFDWMGFAAVAITTSTLILLTTWGGSEYEWTSPTILSMAAVVIVGALLTVFIESRASQPLIPVQLFKNRNMVLTTLAGTVLGLAMMGVLGYMPTYLQMVHTLTPTEAGLMMIPMMVGMIGVSTGVGFIIAKTGNYKYYPIAGLAITAFALWWMTQMTVETSLTGIGVRFLVFGVGLGFVTQVLVLIVQNSFPVSQVGTATAANNFFRQIGSALGASIVGSMFIHKMQNEMATRLPDALASLGKEGAAISQQFQGADAANSLTPHAVAELPDVLRDAILNSYNDGLTPVIGMMVPLAIVAMLILFPLRQERLKETIE

SEQ ID NO: 120 - DNA, 1650 bp, Unknown
  impE2(G64D, I243V, S387T, M413T, N458K)
atggtagctaaaaactccaccccaagcacggccggccacgccagtgctcacactgcggaagaattcccagtggccaatgctgaaatggcaacgccttcagcaatcgacccaaaccacggtaaaaagaccgcggataacgtcggcattatcttcgctgccttgatgctcaccatgctgatgagctctttggaccagatgattttcggttccgctctgccaaccatcgtcggcgagctcggcggcgtggaccagatgagctgggtaatttcagcatttatggtcaccatgaccattgctatgccactagccggtcagctcggtgaccgcatgggccgcaagtgggtctacatctcaggtatctccattttcgttattggctcgacgctcggtggctttgccaatggcatgggcatgctgatcaccggacgtgcaatccagggcttcggtgccggcatcatgatgatttcctcgcagtcgattgtggctgaggttgtctccgcacgtgagcgcggcaagttcatgggtattatgggcggcgtctttggcgtctcctccgtactgggtccagttctcggtggctggttcaccgatggtcccggttggcgttggggcctgtggatcaacattccactgggtctgctggcaattattgtctgcgctttcgtactgaagctgcgcgtgggcgagcaaggctttaagggctttgactggatgggttttgcggccgtcgcaatcacgaccagcaccctgattctgctcaccacttggggcggaagcgaatacgagtggacttccccaactattttgtccatggctgccgtagtcatcgtcggcgcgctgctcaccgtgttcattgagtcgcgtgcatcccagccgctgatcccggttcagctatttaagaaccgcaacatggttttgaccaccctcgccggtactgttttgggtctggccatgatgggcgtgctcggctacatgccaacctacctgcagatggtgcacaccctgacgccaactgaagcaggcttgatgatgatcccgatgatggtcggcatgatcggtgtctccactggtgttggcttcatcatcgctaagaccggcaactacaagtactaccccatcgcgggcctggccatcacggcgtttgctttgtggtggatgacccagatgaccgttgagacttcattgaccggtatcggagttcgcttccttgtattcggtgtcggcttgggctttgtcacgcaggtactggtgctgattgttcaaaactccttccctgtatcgcaggtcggtactgccacggcggctaataacttcttccgccagattggttcggcattgggtgcttccatcgtgggttcgatgttcattcacaaaatgcagaatgagatggctacccgtttgcctgatgcccttgcatcgttgggcaaggaaggcgccgctatttcgcagcagttccaaggtgcagatgccgccaactccttgactccgcacgcagtcgcagagcttcccgatgtcctccgtgacgctatcttaaattcctacaatgacggtctgacccccgtgattggcatgatggtgccactggccattgttgcaatgctgattttgttcccactgcgccaagagcgcttgaaggaaaccatcgaataa

SEQ ID NO: 121 - protein, 549 aa, Unknown
  impE2(G64D, S387T, F405Y, M413T, N458K)
MVAKNSTPSTAGHASAHTAEEFPVANAEMATPSAIDPNHGKKTADNVGIIFAALMLTMLMSSLDQMIFGSALPTIVGELGGVDQMSWVISAFMVTMTIAMPLAGQLGDRMGRKWVYISGISIFVIGSTLGGFANGMGMLITGRAIQGFGAGIMMISSQSIVAEVVSARERGKFMGIMGGVFGVSSVLGPVLGGWFTDGPGWRWGLWINIPLGLLAIIVCAFVLKLRVGEQGFKGFDWMGFAAIAITTSTLILLTTWGGSEYEWTSPTILSMAAVVIVGALLTVFIESRASQPLIPVQLFKNRNMVLTTLAGTVLGLAMMGVLGYMPTYLQMVHTLTPTEAGLMMIPMMVGMIGVSTGVGFIIAKTGNYKYYPIAGLAITAFALWWMTQMTVETSLTGIGVRFLVYGVGLGFVTQVLVLIVQNSFPVSQVGTATAANNFFRQIGSALGASIVGSMFIHKMQNEMATRLPDALASLGKEGAAISQQFQGADAANSLTPHAVAELPDVLRDAILNSYNDGLTPVIGMMVPLAIVAMLILFPLRQERLKETIE

SEQ ID NO: 122 - DNA, 1650 bp, Unknown
  impE2(G64D, S387T, F405Y, M413T, N458K)
atggtagctaaaaactccaccccaagcacggccggccacgccagtgctcacactgcggaagaattcccagtggccaatgctgaaatggcaacgccttcagcaatcgacccaaaccacggtaaaaagaccgcggataacgtcggcattatcttcgctgccttgatgctcaccatgctgatgagctctttggaccagatgattttcggttccgctctgccaaccatcgtcggcgagctcggcggcgtggaccagatgagctgggtaatttcagcatttatggtcaccatgaccattgctatgccactagccggtcagctcggtgaccgcatgggccgcaagtgggtctacatctcaggtatctccattttcgttattggctcgacgctcggtggctttgccaatggcatgggcatgctgatcaccggacgtgcaatccagggcttcggtgccggcatcatgatgatttcctcgcagtcgattgtggctgaggttgtctccgcacgtgagcgcggcaagttcatgggtattatgggcggcgtctttggcgtctcctccgtactgggtccagttctcggtggctggttcaccgatggtcccggttggcgttggggcctgtggatcaacattccactgggtctgctggcaattattgtctgcgctttcgtactgaagctgcgcgtgggcgagcaaggctttaagggctttgactggatgggttttgcggccatcgcaatcacgaccagcaccctgattctgctcaccacttggggcggaagcgaatacgagtggacttccccaactattttgtccatggctgccgtagtcatcgtcggcgcgctgctcaccgtgttcattgagtcgcgtgcatcccagccgctgatcccggttcagctatttaagaaccgcaacatggttttgaccaccctcgccggtactgttttgggtctggccatgatgggcgtgctcggctacatgccaacctacctgcagatggtgcacaccctgacgccaactgaagcaggcttgatgatgatcccgatgatggtcggcatgatcggtgtctccactggtgttggcttcatcatcgctaagaccggcaactacaagtactaccccatcgcgggcctggccatcacggcgtttgctttgtggtggatgacccagatgaccgttgagacttcattgaccggtatcggagttcgcttccttgtatacggtgtcggcttgggctttgtcacgcaggtactggtgctgattgttcaaaactccttccctgtatcgcaggtcggtactgccacggcggctaataacttcttccgccagattggttcggcattgggtgcttccatcgtgggttcgatgttcattcacaaaatgcagaatgagatggctacccgtttgcctgatgcccttgcatcgttgggcaaggaaggcgccgctatttcgcagcagttccaaggtgcagatgccgccaactccttgactccgcacgcagtcgcagagcttcccgatgtcctccgtgacgctatcttaaattcctacaatgacggtctgacccccgtgattggcatgatggtgccactggccattgttgcaatgctgattttgttcccactgcgccaagagcgcttgaaggaaaccatcgaataa

SEQ ID NO: 123 - protein, 549 aa, Unknown
  impE2(G64D, F123C, S387T, M413T, N458K)
MVAKNSTPSTAGHASAHTAEEFPVANAEMATPSAIDPNHGKKTADNVGIIFAALMLTMLMSSLDQMIFGSALPTIVGELGGVDQMSWVISAFMVTMTIAMPLAGQLGDRMGRKWVYISGISICVIGSTLGGFANGMGMLITGRAIQGFGAGIMMISSQSIVAEVVSARERGKFMGIMGGVFGVSSVLGPVLGGWFTDGPGWRWGLWINIPLGLLAIIVCAFVLKLRVGEQGFKGFDWMGFAAIAITTSTLILLTTWGGSEYEWTSPTILSMAAVVIVGALLTVFIESRASQPLIPVQLFKNRNMVLTTLAGTVLGLAMMGVLGYMPTYLQMVHTLTPTEAGLMMIPMMVGMIGVSTGVGFIIAKTGNYKYYPIAGLAITAFALWWMTQMTVETSLTGIGVRFLVFGVGLGFVTQVLVLIVQNSFPVSQVGTATAANNFFRQIGSALGASIVGSMFIHKMQNEMATRLPDALASLGKEGAAISQQFQGADAANSLTPHAVAELPDVLRDAILNSYNDGLTPVIGMMVPLAIVAMLILFPLRQERLKETIE

SEQ ID NO: 124 - DNA, 1650 bp, Unknown
  impE2(G64D, F123C, S387T, M413T, N458K)
atggtagctaaaaactccaccccaagcacggccggccacgccagtgctcacactgcggaagaattcccagtggccaatgctgaaatggcaacgccttcagcaatcgacccaaaccacggtaaaaagaccgcggataacgtcggcattatcttcgctgccttgatgctcaccatgctgatgagctctttggaccagatgattttcggttccgctctgccaaccatcgtcggcgagctcggcggcgtggaccagatgagctgggtaatttcagcatttatggtcaccatgaccattgctatgccactagccggtcagctcggtgaccgcatgggccgcaagtgggtctacatctcaggtatctccatttgcgttattggctcgacgctcggtggctttgccaatggcatgggcatgctgatcaccggacgtgcaatccagggcttcggtgccggcatcatgatgatttcctcgcagtcgattgtggctgaggttgtctccgcacgtgagcgcggcaagttcatgggtattatgggcggcgtctttggcgtctcctccgtactgggtccagttctcggtggctggttcaccgatggtcccggttggcgttggggcctgtggatcaacattccactgggtctgctggcaattattgtctgcgctttcgtactgaagctgcgcgtgggcgagcaaggctttaagggctttgactggatgggttttgcggccatcgcaatcacgaccagcaccctgattctgctcaccacttggggcggaagcgaatacgagtggacttccccaactattttgtccatggctgccgtagtcatcgtcggcgcgctgctcaccgtgttcattgagtcgcgtgcatcccagccgctgatcccggttcagctatttaagaaccgcaacatggttttgaccaccctcgccggtactgttttgggtctggccatgatgggcgtgctcggctacatgccaacctacctgcagatggtgcacaccctgacgccaactgaagcaggcttgatgatgatcccgatgatggtcggcatgatcggtgtctccactggtgttggcttcatcatcgctaagaccggcaactacaagtactaccccatcgcgggcctggccatcacggcgtttgctttgtggtggatgacccagatgaccgttgagacttcattgaccggtatcggagttcgcttccttgtattcggtgtcggcttgggctttgtcacgcaggtactggtgctgattgttcaaaactccttccctgtatcgcaggtcggtactgccacggcggctaataacttcttccgccagattggttcggcattgggtgcttccatcgtgggttcgatgttcattcacaaaatgcagaatgagatggctacccgtttgcctgatgcccttgcatcgttgggcaaggaaggcgccgctatttcgcagcagttccaaggtgcagatgccgccaactccttgactccgcacgcagtcgcagagcttcccgatgtcctccgtgacgctatcttaaattcctacaatgacggtctgacccccgtgattggcatgatggtgccactggccattgttgcaatgctgattttgttcccactgcgccaagagcgcttgaaggaaaccatcgaataa

SEQ ID NO: 125 - protein, 549 aa, Unknown
  impE2(G64D, I243V, S387T, F405Y, M413T, N458K)
MVAKNSTPSTAGHASAHTAEEFPVANAEMATPSAIDPNHGKKTADNVGIIFAALMLTMLMSSLDQMIFGSALPTIVGELGGVDQMSWVISAFMVTMTIAMPLAGQLGDRMGRKWVYISGISIFVIGSTLGGFANGMGMLITGRAIQGFGAGIMMISSQSIVAEVVSARERGKFMGIMGGVFGVSSVLGPVLGGWFTDGPGWRWGLWINIPLGLLAIIVCAFVLKLRVGEQGFKGFDWMGFAAVAITTSTLILLTTWGGSEYEWTSPTILSMAAVVIVGALLTVFIESRASQPLIPVQLFKNRNMVLTTLAGTVLGLAMMGVLGYMPTYLQMVHTLTPTEAGLMMIPMMVGMIGVSTGVGFIIAKTGNYKYYPIAGLAITAFALWWMTQMTVETSLTGIGVRFLVYGVGLGFVTQVLVLIVQNSFPVSQVGTATAANNFFRQIGSALGASIVGSMFIHKMQNEMATRLPDALASLGKEGAAISQQFQGADAANSLTPHAVAELPDVLRDAILNSYNDGLTPVIGMMVPLAIVAMLILFPLRQERLKETIE

SEQ ID NO: 126 - DNA, 1650 bp, Unknown
  impE2(G64D, I243V, S387T, F405Y, M413T, N458K)
atggtagctaaaaactccaccccaagcacggccggccacgccagtgctcacactgcggaagaattcccagtggccaatgctgaaatggcaacgccttcagcaatcgacccaaaccacggtaaaaagaccgcggataacgtcggcattatcttcgctgccttgatgctcaccatgctgatgagctctttggaccagatgattttcggttccgctctgccaaccatcgtcggcgagctcggcggcgtggaccagatgagctgggtaatttcagcatttatggtcaccatgaccattgctatgccactagccggtcagctcggtgaccgcatgggccgcaagtgggtctacatctcaggtatctccattttcgttattggctcgacgctcggtggctttgccaatggcatgggcatgctgatcaccggacgtgcaatccagggcttcggtgccggcatcatgatgatttcctcgcagtcgattgtggctgaggttgtctccgcacgtgagcgcggcaagttcatgggtattatgggcggcgtctttggcgtctcctccgtactgggtccagttctcggtggctggttcaccgatggtcccggttggcgttggggcctgtggatcaacattccactgggtctgctggcaattattgtctgcgctttcgtactgaagctgcgcgtgggcgagcaaggctttaagggctttgactggatgggttttgcggccgtcgcaatcacgaccagcaccctgattctgctcaccacttggggcggaagcgaatacgagtggacttccccaactattttgtccatggctgccgtagtcatcgtcggcgcgctgctcaccgtgttcattgagtcgcgtgcatcccagccgctgatcccggttcagctatttaagaaccgcaacatggttttgaccaccctcgccggtactgttttgggtctggccatgatgggcgtgctcggctacatgccaacctacctgcagatggtgcacaccctgacgccaactgaagcaggcttgatgatgatcccgatgatggtcggcatgatcggtgtctccactggtgttggcttcatcatcgctaagaccggcaactacaagtactaccccatcgcgggcctggccatcacggcgtttgctttgtggtggatgacccagatgaccgttgagacttcattgaccggtatcggagttcgcttccttgtatacggtgtcggcttgggctttgtcacgcaggtactggtgctgattgttcaaaactccttccctgtatcgcaggtcggtactgccacggcggctaataacttcttccgccagattggttcggcattgggtgcttccatcgtgggttcgatgttcattcacaaaatgcagaatgagatggctacccgtttgcctgatgcccttgcatcgttgggcaaggaaggcgccgctatttcgcagcagttccaaggtgcagatgccgccaactccttgactccgcacgcagtcgcagagcttcccgatgtcctccgtgacgctatcttaaattcctacaatgacggtctgacccccgtgattggcatgatggtgccactggccattgttgcaatgctgattttgttcccactgcgccaagagcgcttgaaggaaaccatcgaataa

SEQ ID NO: 127 - protein, 549 aa, Unknown
  impE2(G64D, F123C, I243V, S387T, F405Y, M413T, N458K)
MVAKNSTPSTAGHASAHTAEEFPVANAEMATPSAIDPNHGKKTADNVGIIFAALMLTMLMSSLDQMIFGSALPTIVGELGGVDQMSWVISAFMVTMTIAMPLAGQLGDRMGRKWVYISGISICVIGSTLGGFANGMGMLITGRAIQGFGAGIMMISSQSIVAEVVSARERGKFMGIMGGVFGVSSVLGPVLGGWFTDGPGWRWGLWINIPLGLLAIIVCAFVLKLRVGEQGFKGFDWMGFAAVAITTSTLILLTTWGGSEYEWTSPTILSMAAVVIVGALLTVFIESRASQPLIPVQLFKNRNMVLTTLAGTVLGLAMMGVLGYMPTYLQMVHTLTPTEAGLMMIPMMVGMIGVSTGVGFIIAKTGNYKYYPIAGLAITAFALWWMTQMTVETSLTGIGVRFLVYGVGLGFVTQVLVLIVQNSFPVSQVGTATAANNFFRQIGSALGASIVGSMFIHKMQNEMATRLPDALASLGKEGAAISQQFQGADAANSLTPHAVAELPDVLRDAILNSYNDGLTPVIGMMVPLAIVAMLILFPLRQERLKETIE

SEQ ID NO: 128 - DNA, 1650 bp, Unknown
  impE2(G64D, F123C, I243V, S387T, F405Y, M413T, N458K)
atggtagctaaaaactccaccccaagcacggccggccacgccagtgctcacactgcggaagaattcccagtggccaatgctgaaatggcaacgccttcagcaatcgacccaaaccacggtaaaaagaccgcggataacgtcggcattatcttcgctgccttgatgctcaccatgctgatgagctctttggaccagatgattttcggttccgctctgccaaccatcgtcggcgagctcggcggcgtggaccagatgagctgggtaatttcagcatttatggtcaccatgaccattgctatgccactagccggtcagctcggtgaccgcatgggccgcaagtgggtctacatctcaggtatctccatttgcgttattggctcgacgctcggtggctttgccaatggcatgggcatgctgatcaccggacgtgcaatccagggcttcggtgccggcatcatgatgatttcctcgcagtcgattgtggctgaggttgtctccgcacgtgagcgcggcaagttcatgggtattatgggcggcgtctttggcgtctcctccgtactgggtccagttctcggtggctggttcaccgatggtcccggttggcgttggggcctgtggatcaacattccactgggtctgctggcaattattgtctgcgctttcgtactgaagctgcgcgtgggcgagcaaggctttaagggctttgactggatgggttttgcggccgtcgcaatcacgaccagcaccctgattctgctcaccacttggggcggaagcgaatacgagtggacttccccaactattttgtccatggctgccgtagtcatcgtcggcgcgctgctcaccgtgttcattgagtcgcgtgcatcccagccgctgatcccggttcagctatttaagaaccgcaacatggttttgaccaccctcgccggtactgttttgggtctggccatgatgggcgtgctcggctacatgccaacctacctgcagatggtgcacaccctgacgccaactgaagcaggcttgatgatgatcccgatgatggtcggcatgatcggtgtctccactggtgttggcttcatcatcgctaagaccggcaactacaagtactaccccatcgcgggcctggccatcacggcgtttgctttgtggtggatgacccagatgaccgttgagacttcattgaccggtatcggagttcgcttccttgtatacggtgtcggcttgggctttgtcacgcaggtactggtgctgattgttcaaaactccttccctgtatcgcaggtcggtactgccacggcggctaataacttcttccgccagattggttcggcattgggtgcttccatcgtgggttcgatgttcattcacaaaatgcagaatgagatggctacccgtttgcctgatgcccttgcatcgttgggcaaggaaggcgccgctatttcgcagcagttccaaggtgcagatgccgccaactccttgactccgcacgcagtcgcagagcttcccgatgtcctccgtgacgctatcttaaattcctacaatgacggtctgacccccgtgattggcatgatggtgccactggccattgttgcaatgctgattttgttcccactgcgccaagagcgcttgaaggaaaccatcgaataa

SEQ ID NO: 129 - protein, 549 aa, Unknown
  CJI0323 impE2(S387T, M413T, N458K)
MIAKNSTPSTAGHASAHTAEEFPVANAEMATPSAIDPNHGKKTADNVGIIFAALMLTMLMSSLGQMIFGSALPTIVGELGGVDQMSWVISAFMVTMTIAMPLAGQLGDRMGRKWVYISGISIFVIGSTLGGFANGMGMLITGRAIQGFGAGIMMISSQSIVAEVVSARERGKFMGIMGGVFGVSSVLGPVLGGWFTDGPGWRWGLWINIPLGLLAIIVCAFVLKLRVGEQGFKGFDWMGFAAIAITTSTLILLTTWGGSEYEWTSPTILSMAAVVIVGALLTVFIESRASQPLIPVQLFKNRNMVLTTLAGTVLGLAMMGVLGYMPTYLQMVHTLTPTEAGLMMIPMMVGMIGVSTGVGFIIAKTGNYKYYPIAGLAITAFALWWMTQMTVETSLTGIGVRFLVFGVGLGFVTQVLVLIVQNSFPVSQVGTATAANNFFRQIGSALGASIVGSMFIHKMQNEMATRLPDALASLGKEGAAISQQFQGADAANSLTPHAVAELPDVLRDAILNSYNDGLTPVIGMMVPLAIVAMLILFPLRQERLKETIE

SEQ ID NO: 130 - DNA, 1650 bp, Unknown
  CJI0323 impE2(S387T, M413T, N458K)
atgatagctaaaaactccaccccaagcacggccggccacgccagtgctcacactgcggaagaattcccagtggccaatgctgaaatggcaacgccttcagcaatcgacccaaaccacggtaaaaagaccgcggataacgtcggcattatcttcgctgccttgatgctcaccatgctgatgagctctttggggcagatgattttcggttccgctctgccaaccatcgtcggcgagctcggcggcgtggaccagatgagctgggtaatttcagcatttatggtcaccatgaccattgctatgccactagccggtcagctcggtgaccgcatgggccgcaagtgggtctacatctcaggtatctccattttcgttattggctcgacgctcggtggctttgccaatggcatgggcatgctgatcaccggacgtgcaatccagggcttcggtgccggcatcatgatgatttcctcgcagtcgattgtggctgaggttgtctccgcacgtgagcgcggcaagttcatgggtattatgggcggcgtctttggcgtctcctccgtactgggtccagttctcggtggctggttcaccgatggtcccggttggcgttggggcctgtggatcaacattccactgggtctgctggcaattattgtctgcgctttcgtactgaagctgcgcgtgggcgagcaaggctttaagggctttgactggatgggttttgcggccatcgcaatcacgaccagcaccctgattctgctcaccacttggggcggaagcgaatacgagtggacttccccaactattttgtccatggctgccgtagtcatcgtcggcgcgctgctcaccgtgttcattgagtcgcgtgcatcccagccgctgatcccggttcagctatttaagaaccgcaacatggttttgaccaccctcgccggtactgttttgggtctggccatgatgggcgtgctcggctacatgccaacctacctgcagatggtgcacaccctgacgccaactgaagcaggcttgatgatgatcccgatgatggtcggcatgatcggtgtctccactggtgttggcttcatcatcgctaagaccggcaactacaagtactaccccatcgcgggcctggccatcacggcgtttgctttgtggtggatgacccagatgaccgttgagacttcattgaccggtatcggagttcgcttccttgtattcggtgtcggcttgggctttgtcacgcaggtactggtgctgattgttcaaaactccttccctgtatcgcaggtcggtactgccacggcggctaataacttcttccgccagattggttcggcattgggtgcttccatcgtgggttcgatgttcattcacaaaatgcagaatgagatggctacccgtttgcctgatgcccttgcatcgttgggcaaggaaggcgccgctatttcgcagcagttccaaggtgcagatgccgccaactccttgactccgcacgcagtcgcagagcttcccgatgtcctccgtgacgctatcttaaattcctacaatgacggtctgacccccgtgattggcatgatggtgccactggccattgttgcaatgctgattttgttcccactgcgccaagagcgcttgaaggaaaccatcgaataa

SEQ ID NO: 131 - protein, 549 aa, Unknown
  CJI0323 impE2(G64D, S387T, M413T, N458K)
MIAKNSTPSTAGHASAHTAEEFPVANAEMATPSAIDPNHGKKTADNVGIIFAALMLTMLMSSLDQMIFGSALPTIVGELGGVDQMSWVISAFMVTMTIAMPLAGQLGDRMGRKWVYISGISIFVIGSTLGGFANGMGMLITGRAIQGFGAGIMMISSQSIVAEVVSARERGKFMGIMGGVFGVSSVLGPVLGGWFTDGPGWRWGLWINIPLGLLAIIVCAFVLKLRVGEQGFKGFDWMGFAAIAITTSTLILLTTWGGSEYEWTSPTILSMAAVVIVGALLTVFIESRASQPLIPVQLFKNRNMVLTTLAGTVLGLAMMGVLGYMPTYLQMVHTLTPTEAGLMMIPMMVGMIGVSTGVGFIIAKTGNYKYYPIAGLAITAFALWWMTQMTVETSLTGIGVRFLVFGVGLGFVTQVLVLIVQNSFPVSQVGTATAANNFFRQIGSALGASIVGSMFIHKMQNEMATRLPDALASLGKEGAAISQQFQGADAANSLTPHAVAELPDVLRDAILNSYNDGLTPVIGMMVPLAIVAMLILFPLRQERLKETIE

SEQ ID NO: 132 - DNA, 1650 bp, Unknown
  CJI0323 impE2(G64D, S387T, M413T, N458K)
atgatagctaaaaactccaccccaagcacggccggccacgccagtgctcacactgcggaagaattcccagtggccaatgctgaaatggcaacgccttcagcaatcgacccaaaccacggtaaaaagaccgcggataacgtcggcattatcttcgctgccttgatgctcaccatgctgatgagctctttggaccagatgattttcggttccgctctgccaaccatcgtcggcgagctcggcggcgtggaccagatgagctgggtaatttcagcatttatggtcaccatgaccattgctatgccactagccggtcagctcggtgaccgcatgggccgcaagtgggtctacatctcaggtatctccattttcgttattggctcgacgctcggtggctttgccaatggcatgggcatgctgatcaccggacgtgcaatccagggcttcggtgccggcatcatgatgatttcctcgcagtcgattgtggctgaggttgtctccgcacgtgagcgcggcaagttcatgggtattatgggcggcgtctttggcgtctcctccgtactgggtccagttctcggtggctggttcaccgatggtcccggttggcgttggggcctgtggatcaacattccactgggtctgctggcaattattgtctgcgctttcgtactgaagctgcgcgtgggcgagcaaggctttaagggctttgactggatgggttttgcggccatcgcaatcacgaccagcaccctgattctgctcaccacttggggcggaagcgaatacgagtggacttccccaactattttgtccatggctgccgtagtcatcgtcggcgcgctgctcaccgtgttcattgagtcgcgtgcatcccagccgctgatcccggttcagctatttaagaaccgcaacatggttttgaccaccctcgccggtactgttttgggtctggccatgatgggcgtgctcggctacatgccaacctacctgcagatggtgcacaccctgacgccaactgaagcaggcttgatgatgatcccgatgatggtcggcatgatcggtgtctccactggtgttggcttcatcatcgctaagaccggcaactacaagtactaccccatcgcgggcctggccatcacggcgtttgctttgtggtggatgacccagatgaccgttgagacttcattgaccggtatcggagttcgcttccttgtattcggtgtcggcttgggctttgtcacgcaggtactggtgctgattgttcaaaactccttccctgtatcgcaggtcggtactgccacggcggctaataacttcttccgccagattggttcggcattgggtgcttccatcgtgggttcgatgttcattcacaaaatgcagaatgagatggctacccgtttgcctgatgcccttgcatcgttgggcaaggaaggcgccgctatttcgcagcagttccaaggtgcagatgccgccaactccttgactccgcacgcagtcgcagagcttcccgatgtcctccgtgacgctatcttaaattcctacaatgacggtctgacccccgtgattggcatgatggtgccactggccattgttgcaatgctgattttgttcccactgcgccaagagcgcttgaaggaaaccatcgaataa

SEQ ID NO: 133 - protein, 549 aa, Unknown
  CJI0323 impE2(G64D, F123C)
MIAKNSTPSTAGHASAHTAEEFPVANAEMATPSAIDPNHGKKTADNVGIIFAALMLTMLMSSLDQMIFGSALPTIVGELGGVDQMSWVISAFMVTMTIAMPLAGQLGDRMGRKWVYISGISICVIGSTLGGFANGMGMLITGRAIQGFGAGIMMISSQSIVAEVVSARERGKFMGIMGGVFGVSSVLGPVLGGWFTDGPGWRWGLWINIPLGLLAIIVCAFVLKLRVGEQGFKGFDWMGFAAIAITTSTLILLTTWGGSEYEWTSPTILSMAAVVIVGALLTVFIESRASQPLIPVQLFKNRNMVLTTLAGTVLGLAMMGVLGYMPTYLQMVHTLTPTEAGLMMIPMMVGMIGVSTGVGFIIAKTGNYKYYPIAGLAITAFALWWMSQMTVETSLTGIGVRFLVFGVGLGFVMQVLVLIVQNSFPVSQVGTATAANNFFRQIGSALGASIVGSMFIHNMQNEMATRLPDALASLGKEGAAISQQFQGADAANSLTPHAVAELPDVLRDAILNSYNDGLTPVIGMMVPLAIVAMLILFPLRQERLKETIE

SEQ ID NO: 134 - DNA, 1650 bp, Unknown
  CJI0323 impE2(G64D, F123C)
atgatagctaaaaactccaccccaagcacggccggccacgccagtgctcacactgcggaagaattcccagtggccaatgctgaaatggcaacgccttcagcaatcgacccaaaccacggtaaaaagaccgcggataacgtcggcattatcttcgctgccttgatgctcaccatgctgatgagctctttggaccagatgattttcggttccgctctgccaaccatcgtcggcgagctcggcggcgtggaccagatgagctgggtaatttcagcatttatggtcaccatgaccattgctatgccactagccggtcagctcggtgaccgcatgggccgcaagtgggtctacatctcaggtatctccatttgcgttattggctcgacgctcggtggctttgccaatggcatgggcatgctgatcaccggacgtgcaatccagggcttcggtgccggcatcatgatgatttcctcgcagtcgattgtggctgaggttgtctccgcacgtgagcgcggcaagttcatgggtattatgggcggcgtctttggcgtctcctccgtactgggtccagttctcggtggctggttcaccgatggtcccggttggcgttggggcctgtggatcaacattccactgggtctgctggcaattattgtctgcgctttcgtactgaagctgcgcgtgggcgagcaaggctttaagggctttgactggatgggttttgcggccatcgcaatcacgaccagcaccctgattctgctcaccacttggggcggaagcgaatacgagtggacttccccaactattttgtccatggctgccgtagtcatcgtcggcgcgctgctcaccgtgttcattgagtcgcgtgcatcccagccgctgatcccggttcagctatttaagaaccgcaacatggttttgaccaccctcgccggtactgttttgggtctggccatgatgggcgtgctcggctacatgccaacctacctgcagatggtgcacaccctgacgccaactgaagcaggcttgatgatgatcccgatgatggtcggcatgatcggtgtctccactggtgttggcttcatcatcgctaagaccggcaactacaagtactaccccatcgcgggcctggccatcacggcgtttgctttgtggtggatgtcccagatgaccgttgagacttcattgaccggtatcggagttcgcttccttgtattcggtgtcggcttgggctttgtcatgcaggtactggtgctgattgttcaaaactccttccctgtatcgcaggtcggtactgccacggcggctaataacttcttccgccagattggttcggcattgggtgcttccatcgtgggttcgatgttcattcacaatatgcagaatgagatggctacccgtttgcctgatgcccttgcatcgttgggcaaggaaggcgccgctatttcgcagcagttccaaggtgcagatgccgccaactccttgactccgcacgcagtcgcagagcttcccgatgtcctccgtgacgctatcttaaattcctacaatgacggtctgacccccgtgattggcatgatggtgccactggccattgttgcaatgctgattttgttcccactgcgccaagagcgcttgaaggaaaccatcgaataa

SEQ ID NO: 135 - protein, 549 aa, Unknown
  CJI0323 impE2(G64D, I243V)
MIAKNSTPSTAGHASAHTAEEFPVANAEMATPSAIDPNHGKKTADNVGIIFAALMLTMLMSSLDQMIFGSALPTIVGELGGVDQMSWVISAFMVTMTIAMPLAGQLGDRMGRKWVYISGISIFVIGSTLGGFANGMGMLITGRAIQGFGAGIMMISSQSIVAEVVSARERGKFMGIMGGVFGVSSVLGPVLGGWFTDGPGWRWGLWINIPLGLLAIIVCAFVLKLRVGEQGFKGFDWMGFAAVAITTSTLILLTTWGGSEYEWTSPTILSMAAVVIVGALLTVFIESRASQPLIPVQLFKNRNMVLTTLAGTVLGLAMMGVLGYMPTYLQMVHTLTPTEAGLMMIPMMVGMIGVSTGVGFIIAKTGNYKYYPIAGLAITAFALWWMSQMTVETSLTGIGVRFLVFGVGLGFVMQVLVLIVQNSFPVSQVGTATAANNFFRQIGSALGASIVGSMFIHNMQNEMATRLPDALASLGKEGAAISQQFQGADAANSLTPHAVAELPDVLRDAILNSYNDGLTPVIGMMVPLAIVAMLILFPLRQERLKETIE

SEQ ID NO: 136 - DNA, 1650 bp, Unknown
  CJI0323 impE2(G64D, I243V)
atgatagctaaaaactccaccccaagcacggccggccacgccagtgctcacactgcggaagaattcccagtggccaatgctgaaatggcaacgccttcagcaatcgacccaaaccacggtaaaaagaccgcggataacgtcggcattatcttcgctgccttgatgctcaccatgctgatgagctctttggaccagatgattttcggttccgctctgccaaccatcgtcggcgagctcggcggcgtggaccagatgagctgggtaatttcagcatttatggtcaccatgaccattgctatgccactagccggtcagctcggtgaccgcatgggccgcaagtgggtctacatctcaggtatctccattttcgttattggctcgacgctcggtggctttgccaatggcatgggcatgctgatcaccggacgtgcaatccagggcttcggtgccggcatcatgatgatttcctcgcagtcgattgtggctgaggttgtctccgcacgtgagcgcggcaagttcatgggtattatgggcggcgtctttggcgtctcctccgtactgggtccagttctcggtggctggttcaccgatggtcccggttggcgttggggcctgtggatcaacattccactgggtctgctggcaattattgtctgcgctttcgtactgaagctgcgcgtgggcgagcaaggctttaagggctttgactggatgggttttgcggccgtcgcaatcacgaccagcaccctgattctgctcaccacttggggcggaagcgaatacgagtggacttccccaactattttgtccatggctgccgtagtcatcgtcggcgcgctgctcaccgtgttcattgagtcgcgtgcatcccagccgctgatcccggttcagctatttaagaaccgcaacatggttttgaccaccctcgccggtactgttttgggtctggccatgatgggcgtgctcggctacatgccaacctacctgcagatggtgcacaccctgacgccaactgaagcaggcttgatgatgatcccgatgatggtcggcatgatcggtgtctccactggtgttggcttcatcatcgctaagaccggcaactacaagtactaccccatcgcgggcctggccatcacggcgtttgctttgtggtggatgtcccagatgaccgttgagacttcattgaccggtatcggagttcgcttccttgtattcggtgtcggcttgggctttgtcatgcaggtactggtgctgattgttcaaaactccttccctgtatcgcaggtcggtactgccacggcggctaataacttcttccgccagattggttcggcattgggtgcttccatcgtgggttcgatgttcattcacaatatgcagaatgagatggctacccgtttgcctgatgcccttgcatcgttgggcaaggaaggcgccgctatttcgcagcagttccaaggtgcagatgccgccaactccttgactccgcacgcagtcgcagagcttcccgatgtcctccgtgacgctatcttaaattcctacaatgacggtctgacccccgtgattggcatgatggtgccactggccattgttgcaatgctgattttgttcccactgcgccaagagcgcttgaaggaaaccatcgaataa

SEQ ID NO: 137 - protein, 549 aa, Unknown
  CJI0323 impE2(G64D, F405Y)
MIAKNSTPSTAGHASAHTAEEFPVANAEMATPSAIDPNHGKKTADNVGIIFAALMLTMLMSSLDQMIFGSALPTIVGELGGVDQMSWVISAFMVTMTIAMPLAGQLGDRMGRKWVYISGISIFVIGSTLGGFANGMGMLITGRAIQGFGAGIMMISSQSIVAEVVSARERGKFMGIMGGVFGVSSVLGPVLGGWFTDGPGWRWGLWINIPLGLLAIIVCAFVLKLRVGEQGFKGFDWMGFAAIAITTSTLILLTTWGGSEYEWTSPTILSMAAVVIVGALLTVFIESRASQPLIPVQLFKNRNMVLTTLAGTVLGLAMMGVLGYMPTYLQMVHTLTPTEAGLMMIPMMVGMIGVSTGVGFIIAKTGNYKYYPIAGLAITAFALWWMSQMTVETSLTGIGVRFLVYGVGLGFVMQVLVLIVQNSFPVSQVGTATAANNFFRQIGSALGASIVGSMFIHNMQNEMATRLPDALASLGKEGAAISQQFQGADAANSLTPHAVAELPDVLRDAILNSYNDGLTPVIGMMVPLAIVAMLILFPLRQERLKETIE

SEQ ID NO: 138 - DNA, 1650 bp, Unknown
  CJI0323 impE2(G64D, F405Y)
atgatagctaaaaactccaccccaagcacggccggccacgccagtgctcacactgcggaagaattcccagtggccaatgctgaaatggcaacgccttcagcaatcgacccaaaccacggtaaaaagaccgcggataacgtcggcattatcttcgctgccttgatgctcaccatgctgatgagctctttggaccagatgattttcggttccgctctgccaaccatcgtcggcgagctcggcggcgtggaccagatgagctgggtaatttcagcatttatggtcaccatgaccattgctatgccactagccggtcagctcggtgaccgcatgggccgcaagtgggtctacatctcaggtatctccattttcgttattggctcgacgctcggtggctttgccaatggcatgggcatgctgatcaccggacgtgcaatccagggcttcggtgccggcatcatgatgatttcctcgcagtcgattgtggctgaggttgtctccgcacgtgagcgcggcaagttcatgggtattatgggcggcgtctttggcgtctcctccgtactgggtccagttctcggtggctggttcaccgatggtcccggttggcgttggggcctgtggatcaacattccactgggtctgctggcaattattgtctgcgctttcgtactgaagctgcgcgtgggcgagcaaggctttaagggctttgactggatgggttttgcggccatcgcaatcacgaccagcaccctgattctgctcaccacttggggcggaagcgaatacgagtggacttccccaactattttgtccatggctgccgtagtcatcgtcggcgcgctgctcaccgtgttcattgagtcgcgtgcatcccagccgctgatcccggttcagctatttaagaaccgcaacatggttttgaccaccctcgccggtactgttttgggtctggccatgatgggcgtgctcggctacatgccaacctacctgcagatggtgcacaccctgacgccaactgaagcaggcttgatgatgatcccgatgatggtcggcatgatcggtgtctccactggtgttggcttcatcatcgctaagaccggcaactacaagtactaccccatcgcgggcctggccatcacggcgtttgctttgtggtggatgtcccagatgaccgttgagacttcattgaccggtatcggagttcgcttccttgtatacggtgtcggcttgggctttgtcatgcaggtactggtgctgattgttcaaaactccttccctgtatcgcaggtcggtactgccacggcggctaataacttcttccgccagattggttcggcattgggtgcttccatcgtgggttcgatgttcattcacaatatgcagaatgagatggctacccgtttgcctgatgcccttgcatcgttgggcaaggaaggcgccgctatttcgcagcagttccaaggtgcagatgccgccaactccttgactccgcacgcagtcgcagagcttcccgatgtcctccgtgacgctatcttaaattcctacaatgacggtctgacccccgtgattggcatgatggtgccactggccattgttgcaatgctgattttgttcccactgcgccaagagcgcttgaaggaaaccatcgaataa

SEQ ID NO: 139 - protein, 549 aa, Unknown
  CJI0323 impE2(F123C, I243V, S387T, F405Y, M413T, N458K)
MIAKNSTPSTAGHASAHTAEEFPVANAEMATPSAIDPNHGKKTADNVGIIFAALMLTMLMSSLGQMIFGSALPTIVGELGGVDQMSWVISAFMVTMTIAMPLAGQLGDRMGRKWVYISGISICVIGSTLGGFANGMGMLITGRAIQGFGAGIMMISSQSIVAEVVSARERGKFMGIMGGVFGVSSVLGPVLGGWFTDGPGWRWGLWINIPLGLLAIIVCAFVLKLRVGEQGFKGFDWMGFAAVAITTSTLILLTTWGGSEYEWTSPTILSMAAVVIVGALLTVFIESRASQPLIPVQLFKNRNMVLTTLAGTVLGLAMMGVLGYMPTYLQMVHTLTPTEAGLMMIPMMVGMIGVSTGVGFIIAKTGNYKYYPIAGLAITAFALWWMTQMTVETSLTGIGVRFLVYGVGLGFVTQVLVLIVQNSFPVSQVGTATAANNFFRQIGSALGASIVGSMFIHKMQNEMATRLPDALASLGKEGAAISQQFQGADAANSLTPHAVAELPDVLRDAILNSYNDGLTPVIGMMVPLAIVAMLILFPLRQERLKETIE

SEQ ID NO: 140 - DNA, 1650 bp, Unknown
  CJI0323 impE2(F123C, I243V, S387T, F405Y, M413T, N458K)
atgatagctaaaaactccaccccaagcacggccggccacgccagtgctcacactgcggaagaattcccagtggccaatgctgaaatggcaacgccttcagcaatcgacccaaaccacggtaaaaagaccgcggataacgtcggcattatcttcgctgccttgatgctcaccatgctgatgagctctttggggcagatgattttcggttccgctctgccaaccatcgtcggcgagctcggcggcgtggaccagatgagctgggtaatttcagcatttatggtcaccatgaccattgctatgccactagccggtcagctcggtgaccgcatgggccgcaagtgggtctacatctcaggtatctccatttgcgttattggctcgacgctcggtggctttgccaatggcatgggcatgctgatcaccggacgtgcaatccagggcttcggtgccggcatcatgatgatttcctcgcagtcgattgtggctgaggttgtctccgcacgtgagcgcggcaagttcatgggtattatgggcggcgtctttggcgtctcctccgtactgggtccagttctcggtggctggttcaccgatggtcccggttggcgttggggcctgtggatcaacattccactgggtctgctggcaattattgtctgcgctttcgtactgaagctgcgcgtgggcgagcaaggctttaagggctttgactggatgggttttgcggccgtcgcaatcacgaccagcaccctgattctgctcaccacttggggcggaagcgaatacgagtggacttccccaactattttgtccatggctgccgtagtcatcgtcggcgcgctgctcaccgtgttcattgagtcgcgtgcatcccagccgctgatcccggttcagctatttaagaaccgcaacatggttttgaccaccctcgccggtactgttttgggtctggccatgatgggcgtgctcggctacatgccaacctacctgcagatggtgcacaccctgacgccaactgaagcaggcttgatgatgatcccgatgatggtcggcatgatcggtgtctccactggtgttggcttcatcatcgctaagaccggcaactacaagtactaccccatcgcgggcctggccatcacggcgtttgctttgtggtggatgacccagatgaccgttgagacttcattgaccggtatcggagttcgcttccttgtatacggtgtcggcttgggctttgtcacgcaggtactggtgctgattgttcaaaactccttccctgtatcgcaggtcggtactgccacggcggctaataacttcttccgccagattggttcggcattgggtgcttccatcgtgggttcgatgttcattcacaaaatgcagaatgagatggctacccgtttgcctgatgcccttgcatcgttgggcaaggaaggcgccgctatttcgcagcagttccaaggtgcagatgccgccaactccttgactccgcacgcagtcgcagagcttcccgatgtcctccgtgacgctatcttaaattcctacaatgacggtctgacccccgtgattggcatgatggtgccactggccattgttgcaatgctgattttgttcccactgcgccaagagcgcttgaaggaaaccatcgaataa

SEQ ID NO: 141 - protein, 549 aa, Unknown
  CJI0323 impE2(G64D, S387T)
MIAKNSTPSTAGHASAHTAEEFPVANAEMATPSAIDPNHGKKTADNVGIIFAALMLTMLMSSLDQMIFGSALPTIVGELGGVDQMSWVISAFMVTMTIAMPLAGQLGDRMGRKWVYISGISIFVIGSTLGGFANGMGMLITGRAIQGFGAGIMMISSQSIVAEVVSARERGKFMGIMGGVFGVSSVLGPVLGGWFTDGPGWRWGLWINIPLGLLAIIVCAFVLKLRVGEQGFKGFDWMGFAAIAITTSTLILLTTWGGSEYEWTSPTILSMAAVVIVGALLTVFIESRASQPLIPVQLFKNRNMVLTTLAGTVLGLAMMGVLGYMPTYLQMVHTLTPTEAGLMMIPMMVGMIGVSTGVGFIIAKTGNYKYYPIAGLAITAFALWWMTQMTVETSLTGIGVRFLVFGVGLGFVMQVLVLIVQNSFPVSQVGTATAANNFFRQIGSALGASIVGSMFIHNMQNEMATRLPDALASLGKEGAAISQQFQGADAANSLTPHAVAELPDVLRDAILNSYNDGLTPVIGMMVPLAIVAMLILFPLRQERLKETIE

SEQ ID NO: 142 - DNA, 1650 bp, Unknown
  CJI0323 impE2(G64D, S387T)
atgatagctaaaaactccaccccaagcacggccggccacgccagtgctcacactgcggaagaattcccagtggccaatgctgaaatggcaacgccttcagcaatcgacccaaaccacggtaaaaagaccgcggataacgtcggcattatcttcgctgccttgatgctcaccatgctgatgagctctttggaccagatgattttcggttccgctctgccaaccatcgtcggcgagctcggcggcgtggaccagatgagctgggtaatttcagcatttatggtcaccatgaccattgctatgccactagccggtcagctcggtgaccgcatgggccgcaagtgggtctacatctcaggtatctccattttcgttattggctcgacgctcggtggctttgccaatggcatgggcatgctgatcaccggacgtgcaatccagggcttcggtgccggcatcatgatgatttcctcgcagtcgattgtggctgaggttgtctccgcacgtgagcgcggcaagttcatgggtattatgggcggcgtctttggcgtctcctccgtactgggtccagttctcggtggctggttcaccgatggtcccggttggcgttggggcctgtggatcaacattccactgggtctgctggcaattattgtctgcgctttcgtactgaagctgcgcgtgggcgagcaaggctttaagggctttgactggatgggttttgcggccatcgcaatcacgaccagcaccctgattctgctcaccacttggggcggaagcgaatacgagtggacttccccaactattttgtccatggctgccgtagtcatcgtcggcgcgctgctcaccgtgttcattgagtcgcgtgcatcccagccgctgatcccggttcagctatttaagaaccgcaacatggttttgaccaccctcgccggtactgttttgggtctggccatgatgggcgtgctcggctacatgccaacctacctgcagatggtgcacaccctgacgccaactgaagcaggcttgatgatgatcccgatgatggtcggcatgatcggtgtctccactggtgttggcttcatcatcgctaagaccggcaactacaagtactaccccatcgcgggcctggccatcacggcgtttgctttgtggtggatgacccagatgaccgttgagacttcattgaccggtatcggagttcgcttccttgtattcggtgtcggcttgggctttgtcatgcaggtactggtgctgattgttcaaaactccttccctgtatcgcaggtcggtactgccacggcggctaataacttcttccgccagattggttcggcattgggtgcttccatcgtgggttcgatgttcattcacaatatgcagaatgagatggctacccgtttgcctgatgcccttgcatcgttgggcaaggaaggcgccgctatttcgcagcagttccaaggtgcagatgccgccaactccttgactccgcacgcagtcgcagagcttcccgatgtcctccgtgacgctatcttaaattcctacaatgacggtctgacccccgtgattggcatgatggtgccactggccattgttgcaatgctgattttgttcccactgcgccaagagcgcttgaaggaaaccatcgaataa

SEQ ID NO: 143 - protein, 549 aa, Unknown
  CJI0323 impE2(G64D, M413T)
MIAKNSTPSTAGHASAHTAEEFPVANAEMATPSAIDPNHGKKTADNVGIIFAALMLTMLMSSLDQMIFGSALPTIVGELGGVDQMSWVISAFMVTMTIAMPLAGQLGDRMGRKWVYISGISIFVIGSTLGGFANGMGMLITGRAIQGFGAGIMMISSQSIVAEVVSARERGKFMGIMGGVFGVSSVLGPVLGGWFTDGPGWRWGLWINIPLGLLAIIVCAFVLKLRVGEQGFKGFDWMGFAAIAITTSTLILLTTWGGSEYEWTSPTILSMAAVVIVGALLTVFIESRASQPLIPVQLFKNRNMVLTTLAGTVLGLAMMGVLGYMPTYLQMVHTLTPTEAGLMMIPMMVGMIGVSTGVGFIIAKTGNYKYYPIAGLAITAFALWWMSQMTVETSLTGIGVRFLVFGVGLGFVTQVLVLIVQNSFPVSQVGTATAANNFFRQIGSALGASIVGSMFIHNMQNEMATRLPDALASLGKEGAAISQQFQGADAANSLTPHAVAELPDVLRDAILNSYNDGLTPVIGMMVPLAIVAMLILFPLRQERLKETIE

SEQ ID NO: 144 - DNA, 1650 bp, Unknown
  CJI0323 impE2(G64D, M413T)
atgatagctaaaaactccaccccaagcacggccggccacgccagtgctcacactgcggaagaattcccagtggccaatgctgaaatggcaacgccttcagcaatcgacccaaaccacggtaaaaagaccgcggataacgtcggcattatcttcgctgccttgatgctcaccatgctgatgagctctttggaccagatgattttcggttccgctctgccaaccatcgtcggcgagctcggcggcgtggaccagatgagctgggtaatttcagcatttatggtcaccatgaccattgctatgccactagccggtcagctcggtgaccgcatgggccgcaagtgggtctacatctcaggtatctccattttcgttattggctcgacgctcggtggctttgccaatggcatgggcatgctgatcaccggacgtgcaatccagggcttcggtgccggcatcatgatgatttcctcgcagtcgattgtggctgaggttgtctccgcacgtgagcgcggcaagttcatgggtattatgggcggcgtctttggcgtctcctccgtactgggtccagttctcggtggctggttcaccgatggtcccggttggcgttggggcctgtggatcaacattccactgggtctgctggcaattattgtctgcgctttcgtactgaagctgcgcgtgggcgagcaaggctttaagggctttgactggatgggttttgcggccatcgcaatcacgaccagcaccctgattctgctcaccacttggggcggaagcgaatacgagtggacttccccaactattttgtccatggctgccgtagtcatcgtcggcgcgctgctcaccgtgttcattgagtcgcgtgcatcccagccgctgatcccggttcagctatttaagaaccgcaacatggttttgaccaccctcgccggtactgttttgggtctggccatgatgggcgtgctcggctacatgccaacctacctgcagatggtgcacaccctgacgccaactgaagcaggcttgatgatgatcccgatgatggtcggcatgatcggtgtctccactggtgttggcttcatcatcgctaagaccggcaactacaagtactaccccatcgcgggcctggccatcacggcgtttgctttgtggtggatgtcccagatgaccgttgagacttcattgaccggtatcggagttcgcttccttgtattcggtgtcggcttgggctttgtcacgcaggtactggtgctgattgttcaaaactccttccctgtatcgcaggtcggtactgccacggcggctaataacttcttccgccagattggttcggcattgggtgcttccatcgtgggttcgatgttcattcacaatatgcagaatgagatggctacccgtttgcctgatgcccttgcatcgttgggcaaggaaggcgccgctatttcgcagcagttccaaggtgcagatgccgccaactccttgactccgcacgcagtcgcagagcttcccgatgtcctccgtgacgctatcttaaattcctacaatgacggtctgacccccgtgattggcatgatggtgccactggccattgttgcaatgctgattttgttcccactgcgccaagagcgcttgaaggaaaccatcgaataa

SEQ ID NO: 145 - protein, 549 aa, Unknown
  CJI0323 impE2(G64D, N458K)
MIAKNSTPSTAGHASAHTAEEFPVANAEMATPSAIDPNHGKKTADNVGIIFAALMLTMLMSSLDQMIFGSALPTIVGELGGVDQMSWVISAFMVTMTIAMPLAGQLGDRMGRKWVYISGISIFVIGSTLGGFANGMGMLITGRAIQGFGAGIMMISSQSIVAEVVSARERGKFMGIMGGVFGVSSVLGPVLGGWFTDGPGWRWGLWINIPLGLLAIIVCAFVLKLRVGEQGFKGFDWMGFAAIAITTSTLILLTTWGGSEYEWTSPTILSMAAVVIVGALLTVFIESRASQPLIPVQLFKNRNMVLTTLAGTVLGLAMMGVLGYMPTYLQMVHTLTPTEAGLMMIPMMVGMIGVSTGVGFIIAKTGNYKYYPIAGLAITAFALWWMSQMTVETSLTGIGVRFLVFGVGLGFVMQVLVLIVQNSFPVSQVGTATAANNFFRQIGSALGASIVGSMFIHKMQNEMATRLPDALASLGKEGAAISQQFQGADAANSLTPHAVAELPDVLRDAILNSYNDGLTPVIGMMVPLAIVAMLILFPLRQERLKETIE

SEQ ID NO: 146 - DNA, 1650 bp, Unknown
  CJI0323 impE2(G64D, N458K)
atgatagctaaaaactccaccccaagcacggccggccacgccagtgctcacactgcggaagaattcccagtggccaatgctgaaatggcaacgccttcagcaatcgacccaaaccacggtaaaaagaccgcggataacgtcggcattatcttcgctgccttgatgctcaccatgctgatgagctctttggaccagatgattttcggttccgctctgccaaccatcgtcggcgagctcggcggcgtggaccagatgagctgggtaatttcagcatttatggtcaccatgaccattgctatgccactagccggtcagctcggtgaccgcatgggccgcaagtgggtctacatctcaggtatctccattttcgttattggctcgacgctcggtggctttgccaatggcatgggcatgctgatcaccggacgtgcaatccagggcttcggtgccggcatcatgatgatttcctcgcagtcgattgtggctgaggttgtctccgcacgtgagcgcggcaagttcatgggtattatgggcggcgtctttggcgtctcctccgtactgggtccagttctcggtggctggttcaccgatggtcccggttggcgttggggcctgtggatcaacattccactgggtctgctggcaattattgtctgcgctttcgtactgaagctgcgcgtgggcgagcaaggctttaagggctttgactggatgggttttgcggccatcgcaatcacgaccagcaccctgattctgctcaccacttggggcggaagcgaatacgagtggacttccccaactattttgtccatggctgccgtagtcatcgtcggcgcgctgctcaccgtgttcattgagtcgcgtgcatcccagccgctgatcccggttcagctatttaagaaccgcaacatggttttgaccaccctcgccggtactgttttgggtctggccatgatgggcgtgctcggctacatgccaacctacctgcagatggtgcacaccctgacgccaactgaagcaggcttgatgatgatcccgatgatggtcggcatgatcggtgtctccactggtgttggcttcatcatcgctaagaccggcaactacaagtactaccccatcgcgggcctggccatcacggcgtttgctttgtggtggatgtcccagatgaccgttgagacttcattgaccggtatcggagttcgcttccttgtattcggtgtcggcttgggctttgtcatgcaggtactggtgctgattgttcaaaactccttccctgtatcgcaggtcggtactgccacggcggctaataacttcttccgccagattggttcggcattgggtgcttccatcgtgggttcgatgttcattcacaaaatgcagaatgagatggctacccgtttgcctgatgcccttgcatcgttgggcaaggaaggcgccgctatttcgcagcagttccaaggtgcagatgccgccaactccttgactccgcacgcagtcgcagagcttcccgatgtcctccgtgacgctatcttaaattcctacaatgacggtctgacccccgtgattggcatgatggtgccactggccattgttgcaatgctgattttgttcccactgcgccaagagcgcttgaaggaaaccatcgaataa

SEQ ID NO: 147 - protein, 549 aa, Unknown
  CJI0323 impE2(G64D, I243V, S387T, M413T, N458K)
MIAKNSTPSTAGHASAHTAEEFPVANAEMATPSAIDPNHGKKTADNVGIIFAALMLTMLMSSLDQMIFGSALPTIVGELGGVDQMSWVISAFMVTMTIAMPLAGQLGDRMGRKWVYISGISIFVIGSTLGGFANGMGMLITGRAIQGFGAGIMMISSQSIVAEVVSARERGKFMGIMGGVFGVSSVLGPVLGGWFTDGPGWRWGLWINIPLGLLAIIVCAFVLKLRVGEQGFKGFDWMGFAAVAITTSTLILLTTWGGSEYEWTSPTILSMAAVVIVGALLTVFIESRASQPLIPVQLFKNRNMVLTTLAGTVLGLAMMGVLGYMPTYLQMVHTLTPTEAGLMMIPMMVGMIGVSTGVGFIIAKTGNYKYYPIAGLAITAFALWWMTQMTVETSLTGIGVRFLVFGVGLGFVTQVLVLIVQNSFPVSQVGTATAANNFFRQIGSALGASIVGSMFIHKMQNEMATRLPDALASLGKEGAAISQQFQGADAANSLTPHAVAELPDVLRDAILNSYNDGLTPVIGMMVPLAIVAMLILFPLRQERLKETIE

SEQ ID NO: 148 - DNA, 1650 bp, Unknown
  CJI0323 impE2(G64D, I243V, S387T, M413T, N458K)
atgatagctaaaaactccaccccaagcacggccggccacgccagtgctcacactgcggaagaattcccagtggccaatgctgaaatggcaacgccttcagcaatcgacccaaaccacggtaaaaagaccgcggataacgtcggcattatcttcgctgccttgatgctcaccatgctgatgagctctttggaccagatgattttcggttccgctctgccaaccatcgtcggcgagctcggcggcgtggaccagatgagctgggtaatttcagcatttatggtcaccatgaccattgctatgccactagccggtcagctcggtgaccgcatgggccgcaagtgggtctacatctcaggtatctccattttcgttattggctcgacgctcggtggctttgccaatggcatgggcatgctgatcaccggacgtgcaatccagggcttcggtgccggcatcatgatgatttcctcgcagtcgattgtggctgaggttgtctccgcacgtgagcgcggcaagttcatgggtattatgggcggcgtctttggcgtctcctccgtactgggtccagttctcggtggctggttcaccgatggtcccggttggcgttggggcctgtggatcaacattccactgggtctgctggcaattattgtctgcgctttcgtactgaagctgcgcgtgggcgagcaaggctttaagggctttgactggatgggttttgcggccgtcgcaatcacgaccagcaccctgattctgctcaccacttggggcggaagcgaatacgagtggacttccccaactattttgtccatggctgccgtagtcatcgtcggcgcgctgctcaccgtgttcattgagtcgcgtgcatcccagccgctgatcccggttcagctatttaagaaccgcaacatggttttgaccaccctcgccggtactgttttgggtctggccatgatgggcgtgctcggctacatgccaacctacctgcagatggtgcacaccctgacgccaactgaagcaggcttgatgatgatcccgatgatggtcggcatgatcggtgtctccactggtgttggcttcatcatcgctaagaccggcaactacaagtactaccccatcgcgggcctggccatcacggcgtttgctttgtggtggatgacccagatgaccgttgagacttcattgaccggtatcggagttcgcttccttgtattcggtgtcggcttgggctttgtcacgcaggtactggtgctgattgttcaaaactccttccctgtatcgcaggtcggtactgccacggcggctaataacttcttccgccagattggttcggcattgggtgcttccatcgtgggttcgatgttcattcacaaaatgcagaatgagatggctacccgtttgcctgatgcccttgcatcgttgggcaaggaaggcgccgctatttcgcagcagttccaaggtgcagatgccgccaactccttgactccgcacgcagtcgcagagcttcccgatgtcctccgtgacgctatcttaaattcctacaatgacggtctgacccccgtgattggcatgatggtgccactggccattgttgcaatgctgattttgttcccactgcgccaagagcgcttgaaggaaaccatcgaataa

SEQ ID NO: 149 - protein, 549 aa, Unknown
  CJI0323 impE2(G64D, S387T, F405Y, M413T, N458K)
MIAKNSTPSTAGHASAHTAEEFPVANAEMATPSAIDPNHGKKTADNVGIIFAALMLTMLMSSLDQMIFGSALPTIVGELGGVDQMSWVISAFMVTMTIAMPLAGQLGDRMGRKWVYISGISIFVIGSTLGGFANGMGMLITGRAIQGFGAGIMMISSQSIVAEVVSARERGKFMGIMGGVFGVSSVLGPVLGGWFTDGPGWRWGLWINIPLGLLAIIVCAFVLKLRVGEQGFKGFDWMGFAAIAITTSTLILLTTWGGSEYEWTSPTILSMAAVVIVGALLTVFIESRASQPLIPVQLFKNRNMVLTTLAGTVLGLAMMGVLGYMPTYLQMVHTLTPTEAGLMMIPMMVGMIGVSTGVGFIIAKTGNYKYYPIAGLAITAFALWWMTQMTVETSLTGIGVRFLVYGVGLGFVTQVLVLIVQNSFPVSQVGTATAANNFFRQIGSALGASIVGSMFIHKMQNEMATRLPDALASLGKEGAAISQQFQGADAANSLTPHAVAELPDVLRDAILNSYNDGLTPVIGMMVPLAIVAMLILFPLRQERLKETIE

SEQ ID NO: 150 - DNA, 1650 bp, Unknown
  CJI0323 impE2(G64D, S387T, F405Y, M413T, N458K)
atgatagctaaaaactccaccccaagcacggccggccacgccagtgctcacactgcggaagaattcccagtggccaatgctgaaatggcaacgccttcagcaatcgacccaaaccacggtaaaaagaccgcggataacgtcggcattatcttcgctgccttgatgctcaccatgctgatgagctctttggaccagatgattttcggttccgctctgccaaccatcgtcggcgagctcggcggcgtggaccagatgagctgggtaatttcagcatttatggtcaccatgaccattgctatgccactagccggtcagctcggtgaccgcatgggccgcaagtgggtctacatctcaggtatctccattttcgttattggctcgacgctcggtggctttgccaatggcatgggcatgctgatcaccggacgtgcaatccagggcttcggtgccggcatcatgatgatttcctcgcagtcgattgtggctgaggttgtctccgcacgtgagcgcggcaagttcatgggtattatgggcggcgtctttggcgtctcctccgtactgggtccagttctcggtggctggttcaccgatggtcccggttggcgttggggcctgtggatcaacattccactgggtctgctggcaattattgtctgcgctttcgtactgaagctgcgcgtgggcgagcaaggctttaagggctttgactggatgggttttgcggccatcgcaatcacgaccagcaccctgattctgctcaccacttggggcggaagcgaatacgagtggacttccccaactattttgtccatggctgccgtagtcatcgtcggcgcgctgctcaccgtgttcattgagtcgcgtgcatcccagccgctgatcccggttcagctatttaagaaccgcaacatggttttgaccaccctcgccggtactgttttgggtctggccatgatgggcgtgctcggctacatgccaacctacctgcagatggtgcacaccctgacgccaactgaagcaggcttgatgatgatcccgatgatggtcggcatgatcggtgtctccactggtgttggcttcatcatcgctaagaccggcaactacaagtactaccccatcgcgggcctggccatcacggcgtttgctttgtggtggatgacccagatgaccgttgagacttcattgaccggtatcggagttcgcttccttgtatacggtgtcggcttgggctttgtcacgcaggtactggtgctgattgttcaaaactccttccctgtatcgcaggtcggtactgccacggcggctaataacttcttccgccagattggttcggcattgggtgcttccatcgtgggttcgatgttcattcacaaaatgcagaatgagatggctacccgtttgcctgatgcccttgcatcgttgggcaaggaaggcgccgctatttcgcagcagttccaaggtgcagatgccgccaactccttgactccgcacgcagtcgcagagcttcccgatgtcctccgtgacgctatcttaaattcctacaatgacggtctgacccccgtgattggcatgatggtgccactggccattgttgcaatgctgattttgttcccactgcgccaagagcgcttgaaggaaaccatcgaataa

SEQ ID NO: 151 - protein, 549 aa, Unknown
  CJI0323 impE2(G64D, F123C, S387T, M413T, N458K)
MIAKNSTPSTAGHASAHTAEEFPVANAEMATPSAIDPNHGKKTADNVGIIFAALMLTMLMSSLDQMIFGSALPTIVGELGGVDQMSWVISAFMVTMTIAMPLAGQLGDRMGRKWVYISGISICVIGSTLGGFANGMGMLITGRAIQGFGAGIMMISSQSIVAEVVSARERGKFMGIMGGVFGVSSVLGPVLGGWFTDGPGWRWGLWINIPLGLLAIIVCAFVLKLRVGEQGFKGFDWMGFAAIAITTSTLILLTTWGGSEYEWTSPTILSMAAVVIVGALLTVFIESRASQPLIPVQLFKNRNMVLTTLAGTVLGLAMMGVLGYMPTYLQMVHTLTPTEAGLMMIPMMVGMIGVSTGVGFIIAKTGNYKYYPIAGLAITAFALWWMTQMTVETSLTGIGVRFLVFGVGLGFVTQVLVLIVQNSFPVSQVGTATAANNFFRQIGSALGASIVGSMFIHKMQNEMATRLPDALASLGKEGAAISQQFQGADAANSLTPHAVAELPDVLRDAILNSYNDGLTPVIGMMVPLAIVAMLILFPLRQERLKETIE

SEQ ID NO: 152 - DNA, 1650 bp, Unknown
  CJI0323 impE2(G64D, F123C, S387T, M413T, N458K)
atgatagctaaaaactccaccccaagcacggccggccacgccagtgctcacactgcggaagaattcccagtggccaatgctgaaatggcaacgccttcagcaatcgacccaaaccacggtaaaaagaccgcggataacgtcggcattatcttcgctgccttgatgctcaccatgctgatgagctctttggaccagatgattttcggttccgctctgccaaccatcgtcggcgagctcggcggcgtggaccagatgagctgggtaatttcagcatttatggtcaccatgaccattgctatgccactagccggtcagctcggtgaccgcatgggccgcaagtgggtctacatctcaggtatctccatttgcgttattggctcgacgctcggtggctttgccaatggcatgggcatgctgatcaccggacgtgcaatccagggcttcggtgccggcatcatgatgatttcctcgcagtcgattgtggctgaggttgtctccgcacgtgagcgcggcaagttcatgggtattatgggcggcgtctttggcgtctcctccgtactgggtccagttctcggtggctggttcaccgatggtcccggttggcgttggggcctgtggatcaacattccactgggtctgctggcaattattgtctgcgctttcgtactgaagctgcgcgtgggcgagcaaggctttaagggctttgactggatgggttttgcggccatcgcaatcacgaccagcaccctgattctgctcaccacttggggcggaagcgaatacgagtggacttccccaactattttgtccatggctgccgtagtcatcgtcggcgcgctgctcaccgtgttcattgagtcgcgtgcatcccagccgctgatcccggttcagctatttaagaaccgcaacatggttttgaccaccctcgccggtactgttttgggtctggccatgatgggcgtgctcggctacatgccaacctacctgcagatggtgcacaccctgacgccaactgaagcaggcttgatgatgatcccgatgatggtcggcatgatcggtgtctccactggtgttggcttcatcatcgctaagaccggcaactacaagtactaccccatcgcgggcctggccatcacggcgtttgctttgtggtggatgacccagatgaccgttgagacttcattgaccggtatcggagttcgcttccttgtattcggtgtcggcttgggctttgtcacgcaggtactggtgctgattgttcaaaactccttccctgtatcgcaggtcggtactgccacggcggctaataacttcttccgccagattggttcggcattgggtgcttccatcgtgggttcgatgttcattcacaaaatgcagaatgagatggctacccgtttgcctgatgcccttgcatcgttgggcaaggaaggcgccgctatttcgcagcagttccaaggtgcagatgccgccaactccttgactccgcacgcagtcgcagagcttcccgatgtcctccgtgacgctatcttaaattcctacaatgacggtctgacccccgtgattggcatgatggtgccactggccattgttgcaatgctgattttgttcccactgcgccaagagcgcttgaaggaaaccatcgaataa

SEQ ID NO: 153 - protein, 549 aa, Unknown
  CJI0323 impE2(G64D, I243V, S387T, F405Y, M413T, N458K)
MIAKNSTPSTAGHASAHTAEEFPVANAEMATPSAIDPNHGKKTADNVGIIFAALMLTMLMSSLDQMIFGSALPTIVGELGGVDQMSWVISAFMVTMTIAMPLAGQLGDRMGRKWVYISGISIFVIGSTLGGFANGMGMLITGRAIQGFGAGIMMISSQSIVAEVVSARERGKFMGIMGGVFGVSSVLGPVLGGWFTDGPGWRWGLWINIPLGLLAIIVCAFVLKLRVGEQGFKGFDWMGFAAVAITTSTLILLTTWGGSEYEWTSPTILSMAAVVIVGALLTVFIESRASQPLIPVQLFKNRNMVLTTLAGTVLGLAMMGVLGYMPTYLQMVHTLTPTEAGLMMIPMMVGMIGVSTGVGFIIAKTGNYKYYPIAGLAITAFALWWMTQMTVETSLTGIGVRFLVYGVGLGFVTQVLVLIVQNSFPVSQVGTATAANNFFRQIGSALGASIVGSMFIHKMQNEMATRLPDALASLGKEGAAISQQFQGADAANSLTPHAVAELPDVLRDAILNSYNDGLTPVIGMMVPLAIVAMLILFPLRQERLKETIE

SEQ ID NO: 154 - DNA, 1650 bp, Unknown
  CJI0323 impE2(G64D, I243V, S387T, F405Y, M413T, N458K)
atgatagctaaaaactccaccccaagcacggccggccacgccagtgctcacactgcggaagaattcccagtggccaatgctgaaatggcaacgccttcagcaatcgacccaaaccacggtaaaaagaccgcggataacgtcggcattatcttcgctgccttgatgctcaccatgctgatgagctctttggaccagatgattttcggttccgctctgccaaccatcgtcggcgagctcggcggcgtggaccagatgagctgggtaatttcagcatttatggtcaccatgaccattgctatgccactagccggtcagctcggtgaccgcatgggccgcaagtgggtctacatctcaggtatctccattttcgttattggctcgacgctcggtggctttgccaatggcatgggcatgctgatcaccggacgtgcaatccagggcttcggtgccggcatcatgatgatttcctcgcagtcgattgtggctgaggttgtctccgcacgtgagcgcggcaagttcatgggtattatgggcggcgtctttggcgtctcctccgtactgggtccagttctcggtggctggttcaccgatggtcccggttggcgttggggcctgtggatcaacattccactgggtctgctggcaattattgtctgcgctttcgtactgaagctgcgcgtgggcgagcaaggctttaagggctttgactggatgggttttgcggccgtcgcaatcacgaccagcaccctgattctgctcaccacttggggcggaagcgaatacgagtggacttccccaactattttgtccatggctgccgtagtcatcgtcggcgcgctgctcaccgtgttcattgagtcgcgtgcatcccagccgctgatcccggttcagctatttaagaaccgcaacatggttttgaccaccctcgccggtactgttttgggtctggccatgatgggcgtgctcggctacatgccaacctacctgcagatggtgcacaccctgacgccaactgaagcaggcttgatgatgatcccgatgatggtcggcatgatcggtgtctccactggtgttggcttcatcatcgctaagaccggcaactacaagtactaccccatcgcgggcctggccatcacggcgtttgctttgtggtggatgacccagatgaccgttgagacttcattgaccggtatcggagttcgcttccttgtatacggtgtcggcttgggctttgtcacgcaggtactggtgctgattgttcaaaactccttccctgtatcgcaggtcggtactgccacggcggctaataacttcttccgccagattggttcggcattgggtgcttccatcgtgggttcgatgttcattcacaaaatgcagaatgagatggctacccgtttgcctgatgcccttgcatcgttgggcaaggaaggcgccgctatttcgcagcagttccaaggtgcagatgccgccaactccttgactccgcacgcagtcgcagagcttcccgatgtcctccgtgacgctatcttaaattcctacaatgacggtctgacccccgtgattggcatgatggtgccactggccattgttgcaatgctgattttgttcccactgcgccaagagcgcttgaaggaaaccatcgaataa

SEQ ID NO: 155 - protein, 549 aa, Unknown
  CJI0323 impE2(G64D, F123C, I243V, S387T, F405Y, M413T, N458K)
MIAKNSTPSTAGHASAHTAEEFPVANAEMATPSAIDPNHGKKTADNVGIIFAALMLTMLMSSLDQMIFGSALPTIVGELGGVDQMSWVISAFMVTMTIAMPLAGQLGDRMGRKWVYISGISICVIGSTLGGFANGMGMLITGRAIQGFGAGIMMISSQSIVAEVVSARERGKFMGIMGGVFGVSSVLGPVLGGWFTDGPGWRWGLWINIPLGLLAIIVCAFVLKLRVGEQGFKGFDWMGFAAVAITTSTLILLTTWGGSEYEWTSPTILSMAAVVIVGALLTVFIESRASQPLIPVQLFKNRNMVLTTLAGTVLGLAMMGVLGYMPTYLQMVHTLTPTEAGLMMIPMMVGMIGVSTGVGFIIAKTGNYKYYPIAGLAITAFALWWMTQMTVETSLTGIGVRFLVYGVGLGFVTQVLVLIVQNSFPVSQVGTATAANNFFRQIGSALGASIVGSMFIHKMQNEMATRLPDALASLGKEGAAISQQFQGADAANSLTPHAVAELPDVLRDAILNSYNDGLTPVIGMMVPLAIVAMLILFPLRQERLKETIE

SEQ ID NO: 156 - DNA, 1650 bp, Unknown
  CJI0323 impE2(G64D, F123C, I243V, S387T, F405Y, M413T, N458K)
atgatagctaaaaactccaccccaagcacggccggccacgccagtgctcacactgcggaagaattcccagtggccaatgctgaaatggcaacgccttcagcaatcgacccaaaccacggtaaaaagaccgcggataacgtcggcattatcttcgctgccttgatgctcaccatgctgatgagctctttggaccagatgattttcggttccgctctgccaaccatcgtcggcgagctcggcggcgtggaccagatgagctgggtaatttcagcatttatggtcaccatgaccattgctatgccactagccggtcagctcggtgaccgcatgggccgcaagtgggtctacatctcaggtatctccatttgcgttattggctcgacgctcggtggctttgccaatggcatgggcatgctgatcaccggacgtgcaatccagggcttcggtgccggcatcatgatgatttcctcgcagtcgattgtggctgaggttgtctccgcacgtgagcgcggcaagttcatgggtattatgggcggcgtctttggcgtctcctccgtactgggtccagttctcggtggctggttcaccgatggtcccggttggcgttggggcctgtggatcaacattccactgggtctgctggcaattattgtctgcgctttcgtactgaagctgcgcgtgggcgagcaaggctttaagggctttgactggatgggttttgcggccgtcgcaatcacgaccagcaccctgattctgctcaccacttggggcggaagcgaatacgagtggacttccccaactattttgtccatggctgccgtagtcatcgtcggcgcgctgctcaccgtgttcattgagtcgcgtgcatcccagccgctgatcccggttcagctatttaagaaccgcaacatggttttgaccaccctcgccggtactgttttgggtctggccatgatgggcgtgctcggctacatgccaacctacctgcagatggtgcacaccctgacgccaactgaagcaggcttgatgatgatcccgatgatggtcggcatgatcggtgtctccactggtgttggcttcatcatcgctaagaccggcaactacaagtactaccccatcgcgggcctggccatcacggcgtttgctttgtggtggatgacccagatgaccgttgagacttcattgaccggtatcggagttcgcttccttgtatacggtgtcggcttgggctttgtcacgcaggtactggtgctgattgttcaaaactccttccctgtatcgcaggtcggtactgccacggcggctaataacttcttccgccagattggttcggcattgggtgcttccatcgtgggttcgatgttcattcacaaaatgcagaatgagatggctacccgtttgcctgatgcccttgcatcgttgggcaaggaaggcgccgctatttcgcagcagttccaaggtgcagatgccgccaactccttgactccgcacgcagtcgcagagcttcccgatgtcctccgtgacgctatcttaaattcctacaatgacggtctgacccccgtgattggcatgatggtgccactggccattgttgcaatgctgattttgttcccactgcgccaagagcgcttgaaggaaaccatcgaataa